European Patent Application EP 4 484 449 A1, published January 1, 2025. Title: VEGF-BINDING MOLECULE AND PHARMACEUTICAL USE THEREOF. Applicant: Shanghai Regenelead Therapies Co.,LTD. Application WO. The sequence listing filed with the application follows.

SEQUENCE LISTING (100 sequences)

SEQ ID NO: 1 - protein, 1356 aa, Homo sapiens
  source 1..1356: note = Wild-type VEGFR2
MQSKVLLAVALWLCVETRAASVGLPSVSLDLPRLSIQKDILTIKANTTLQITCRGQRDLDWLWPNNQSGSEQRVEVTECSDGLFCKTLTIPKVIGNDTGAYKCFYRETDLASVIYVYVQDYRSPFIASVSDQHGVVYITENKNKTVVIPCLGSISNLNVSLCARYPEKRFVPDGNRISWDSKKGFTIPSYMISYAGMVFCEAKINDESYQSIMYIVVVVGYRIYDVVLSPSHGIELSVGEKLVLNCTARTELNVGIDFNWEYPSSKHQHKKLVNRDLKTQSGSEMKKFLSTLTIDGVTRSDQGLYTCAASSGLMTKKNSTFVRVHEKPFVAFGSGMESLVEATVGERVRIPAKYLGYPPPEIKWYKNGIPLESNHTIKAGHVLTIMEVSERDTGNYTVILTNPISKEKQSHVVSLVVYVPPQIGEKSLISPVDSYQYGTTQTLTCTVYAIPPPHHIHWYWQLEEECANEPSQAVSVTNPYPCEEWRSVEDFQGGNKIEVNKNQFALIEGKNKTVSTLVIQAANVSALYKCEAVNKVGRGERVISFHVTRGPEITLQPDMQPTEQESVSLWCTADRSTFENLTWYKLGPQPLPIHVGELPTPVCKNLDTLWKLNATMFSNSTNDILIMELKNASLQDQGDYVCLAQDRKTKKRHCVVRQLTVLERVAPTITGNLENQTTSIGESIEVSCTASGNPPPQIMWFKDNETLVEDSGIVLKDGNRNLTIRRVRKEDEGLYTCQACSVLGCAKVEAFFIIEGAQEKTNLEIIILVGTAVIAMFFWLLLVIILRTVKRANGGELKTGYLSIVMDPDELPLDEHCERLPYDASKWEFPRDRLKLGKPLGRGAFGQVIEADAFGIDKTATCRTVAVKMLKEGATHSEHRALMSELKILIHIGHHLNVVNLLGACTKPGGPLMVIVEFCKFGNLSTYLRSKRNEFVPYKTKGARFRQGKDYVGAIPVDLKRRLDSITSSQSSASSGFVEEKSLSDVEEEEAPEDLYKDFLTLEHLICYSFQVAKGMEFLASRKCIHRDLAARNILLSEKNVVKICDFGLARDIYKDPDYVRKGDARLPLKWMAPETIFDRVYTIQSDVWSFGVLLWEIFSLGASPYPGVKIDEEFCRRLKEGTRMRAPDYTTPEMYQTMLDCWHGEPSQRPTFSELVEHLGNLLQANAQQDGKDYIVLPISETLSMEEDSGLSLPTSPVSCMEEEEVCDPKFHYDNTAGISQYLQNSKRKSRPVSVKTFEDIPLEEPEVKVIPDDNQTDSGMVLASEELKTLEDRTKLSPSFGGMVPSKSRESVASEGSNQTSGYQSGYHSDDTDTTVYSSEEAELLKLIEIGVQTGSTAQILQPDSGTTLSSPPV

SEQ ID NO: 2 - protein, 1338 aa, Homo sapiens
  source 1..1338: note = Wild-type VEGFR1
MVSYWDTGVLLCALLSCLLLTGSSSGSKLKDPELSLKGTQHIMQAGQTLHLQCRGEAAHKWSLPEMVSKESERLSITKSACGRNGKQFCSTLTLNTAQANHTGFYSCKYLAVPTSKKKETESAIYIFISDTGRPFVEMYSEIPEIIHMTEGRELVIPCRVTSPNITVTLKKFPLDTLIPDGKRIIWDSRKGFIISNATYKEIGLLTCEATVNGHLYKTNYLTHRQTNTIIDVQISTPRPVKLLRGHTLVLNCTATTPLNTRVQMTWSYPDEKNKRASVRRRIDQSNSHANIFYSVLTIDKMQNKDKGLYTCRVRSGPSFKSVNTSVHIYDKAFITVKHRKQQVLETVAGKRSYRLSMKVKAFPSPEVVWLKDGLPATEKSARYLTRGYSLIIKDVTEEDAGNYTILLSIKQSNVFKNLTATLIVNVKPQIYEKAVSSFPDPALYPLGSRQILTCTAYGIPQPTIKWFWHPCNHNHSEARCDFCSNNEESFILDADSNMGNRIESITQRMAIIEGKNKMASTLVVADSRISGIYICIASNKVGTVGRNISFYITDVPNGFHVNLEKMPTEGEDLKLSCTVNKFLYRDVTWILLRTVNNRTMHYSISKQKMAITKEHSITLNLTIMNVSLQDSGTYACRARNVYTGEEILQKKEITIRDQEAPYLLRNLSDHTVAISSSTTLDCHANGVPEPQITWFKNNHKIQQEPGIILGPGSSTLFIERVTEEDEGVYHCKATNQKGSVESSAYLTVQGTSDKSNLELITLTCTCVAATLFWLLLTLFIRKMKRSSSEIKTDYLSIIMDPDEVPLDEQCERLPYDASKWEFARERLKLGKSLGRGAFGKVVQASAFGIKKSPTCRTVAVKMLKEGATASEYKALMTELKILTHIGHHLNVVNLLGACTKQGGPLMVIVEYCKYGNLSNYLKSKRDLFFLNKDAALHMEPKKEKMEPGLEQGKKPRLDSVTSSESFASSGFQEDKSLSDVEEEEDSDGFYKEPITMEDLISYSFQVARGMEFLSSRKCIHRDLAARNILLSENNVVKICDFGLARDIYKNPDYVRKGDTRLPLKWMAPESIFDKIYSTKSDVWSYGVLLWEIFSLGGSPYPGVQMDEDFCSRLREGMRMRAPEYSTPEIYQIMLDCWHRDPKERPRFAELVEKLGDLLQANVQQDGKDYIPINAILTGNSGFTYSTPAFSEDFFKESISAPKFNSGSSDDVRYVNAFKFMSLERIKTFEELLPNATSMFDDYQGDSSTLLASPMLKRFTWTDSKPKASLKIDLRVTSKSKESGLSDVSRPSFCHSSCGHVSEGKRRFTYDHAELERKIACCSPPPDYNSVVLYSTPPI

SEQ ID NO: 3 - protein, 642 aa, synthetic construct
  source 1..642: note = PR1010 (R1D2-R2D3-linker-R2D2-R2D3-Fc)
SDTGRPFVEMYSEIPEIIHMTEGRELVIPCRVTSPNITVTLKKFPLDTLIPDGKRIIWDSRKGFIISNATYKEIGLLTCEATVNGHLYKTNYLTHRQTNTIIDVVLSPSHGIELSVGEKLVLNCTARTELNVGIDFNWEYPSSKHQHKKLVNRDLKTQSGSEMKKFLSTLTIDGVTRSDQGLYTCAASSGLMTKKNSTFVRVHEKGGGGSSPFIASVSDQHGVVYITENKNKTVVIPCLGSISNLNVSLCARYPEKRFVPDGNRISWDSKKGFTIPSYMISYAGMVFCEAKINDESYQSIMYIVVVVGYRIYDVVLSPSHGIELSVGEKLVLNCTARTELNVGIDFNWEYPSSKHQHKKLVNRDLKTQSGSEMKKFLSTLTIDGVTRSDQGLYTCAASSGLMTKKNSTFVRVHEKDKTHTCPPCPAPEAAGGPSVFLFPPKPKDTLMISRTPEVTCVVVDVSHEDPEVKFNWYVDGVEVHNAKTKPREEQYNSTYRVVSVLTVLHQDWLNGKEYKCKVSNKALPAPIEKTISKAKGQPREPQVYTLPPSREEMTKNQVSLTCLVKGFYPSDIAVEWESNGQPENNYKTTPPVLDSDGSFFLYSKLTVDKSRWQQGNVFSCSVMHEALHNHYTQKSLSLSPGK

SEQ ID NO: 4 - protein, 642 aa, synthetic construct
  source 1..642: note = PR1011 (R2D2-R2D3-linker-R1D2-R2D3-Fc)
SPFIASVSDQHGVVYITENKNKTVVIPCLGSISNLNVSLCARYPEKRFVPDGNRISWDSKKGFTIPSYMISYAGMVFCEAKINDESYQSIMYIVVVVGYRIYDVVLSPSHGIELSVGEKLVLNCTARTELNVGIDFNWEYPSSKHQHKKLVNRDLKTQSGSEMKKFLSTLTIDGVTRSDQGLYTCAASSGLMTKKNSTFVRVHEKGGGGSSDTGRPFVEMYSEIPEIIHMTEGRELVIPCRVTSPNITVTLKKFPLDTLIPDGKRIIWDSRKGFIISNATYKEIGLLTCEATVNGHLYKTNYLTHRQTNTIIDVVLSPSHGIELSVGEKLVLNCTARTELNVGIDFNWEYPSSKHQHKKLVNRDLKTQSGSEMKKFLSTLTIDGVTRSDQGLYTCAASSGLMTKKNSTFVRVHEKDKTHTCPPCPAPEAAGGPSVFLFPPKPKDTLMISRTPEVTCVVVDVSHEDPEVKFNWYVDGVEVHNAKTKPREEQYNSTYRVVSVLTVLHQDWLNGKEYKCKVSNKALPAPIEKTISKAKGQPREPQVYTLPPSREEMTKNQVSLTCLVKGFYPSDIAVEWESNGQPENNYKTTPPVLDSDGSFFLYSKLTVDKSRWQQGNVFSCSVMHEALHNHYTQKSLSLSPGK

SEQ ID NO: 5 - protein, 432 aa, synthetic construct
  source 1..432: note = PR1088 (R2D2-R2D3-Fc)
SPFIASVSDQHGVVYITENKNKTVVIPCLGSISNLNVSLCARYPEKRFVPDGNRISWDSKKGFTIPSYMISYAGMVFCEAKINDESYQSIMYIVVVVGYRIYDVVLSPSHGIELSVGEKLVLNCTARTELNVGIDFNWEYPSSKHQHKKLVNRDLKTQSGSEMKKFLSTLTIDGVTRSDQGLYTCAASSGLMTKKNSTFVRVHEKDKTHTCPPCPAPEAAGGPSVFLFPPKPKDTLMISRTPEVTCVVVDVSHEDPEVKFNWYVDGVEVHNAKTKPREEQYNSTYRVVSVLTVLHQDWLNGKEYKCKVSNKALPAPIEKTISKAKGQPREPQVYTLPPSREEMTKNQVSLTCLVKGFYPSDIAVEWESNGQPENNYKTTPPVLDSDGSFFLYSKLTVDKSRWQQGNVFSCSVMHEALHNHYTQKSLSLSPGK

SEQ ID NO: 6 - protein, 432 aa, synthetic construct
  source 1..432: note = PR1160 (R2D2(C162V)-R2D3-Fc)
SPFIASVSDQHGVVYITENKNKTVVIPCLGSISNLNVSLVARYPEKRFVPDGNRISWDSKKGFTIPSYMISYAGMVFCEAKINDESYQSIMYIVVVVGYRIYDVVLSPSHGIELSVGEKLVLNCTARTELNVGIDFNWEYPSSKHQHKKLVNRDLKTQSGSEMKKFLSTLTIDGVTRSDQGLYTCAASSGLMTKKNSTFVRVHEKDKTHTCPPCPAPEAAGGPSVFLFPPKPKDTLMISRTPEVTCVVVDVSHEDPEVKFNWYVDGVEVHNAKTKPREEQYNSTYRVVSVLTVLHQDWLNGKEYKCKVSNKALPAPIEKTISKAKGQPREPQVYTLPPSREEMTKNQVSLTCLVKGFYPSDIAVEWESNGQPENNYKTTPPVLDSDGSFFLYSKLTVDKSRWQQGNVFSCSVMHEALHNHYTQKSLSLSPGK

SEQ ID NO: 7 - protein, 642 aa, synthetic construct
  source 1..642: note = PR1090 (R1D2-R2D3-linker-R2D2(V135Y)-R2D3-Fc)
SDTGRPFVEMYSEIPEIIHMTEGRELVIPCRVTSPNITVTLKKFPLDTLIPDGKRIIWDSRKGFIISNATYKEIGLLTCEATVNGHLYKTNYLTHRQTNTIIDVVLSPSHGIELSVGEKLVLNCTARTELNVGIDFNWEYPSSKHQHKKLVNRDLKTQSGSEMKKFLSTLTIDGVTRSDQGLYTCAASSGLMTKKNSTFVRVHEKGGGGSSPFIASVSDQHGYVYITENKNKTVVIPCLGSISNLNVSLCARYPEKRFVPDGNRISWDSKKGFTIPSYMISYAGMVFCEAKINDESYQSIMYIVVVVGYRIYDVVLSPSHGIELSVGEKLVLNCTARTELNVGIDFNWEYPSSKHQHKKLVNRDLKTQSGSEMKKFLSTLTIDGVTRSDQGLYTCAASSGLMTKKNSTFVRVHEKDKTHTCPPCPAPEAAGGPSVFLFPPKPKDTLMISRTPEVTCVVVDVSHEDPEVKFNWYVDGVEVHNAKTKPREEQYNSTYRVVSVLTVLHQDWLNGKEYKCKVSNKALPAPIEKTISKAKGQPREPQVYTLPPSREEMTKNQVSLTCLVKGFYPSDIAVEWESNGQPENNYKTTPPVLDSDGSFFLYSKLTVDKSRWQQGNVFSCSVMHEALHNHYTQKSLSLSPGK

SEQ ID NO: 8 - protein, 642 aa, synthetic construct
  source 1..642: note = PR1094(R1D2-R2D3-linker-R2D2(C162V)-R2D3-Fc)
SDTGRPFVEMYSEIPEIIHMTEGRELVIPCRVTSPNITVTLKKFPLDTLIPDGKRIIWDSRKGFIISNATYKEIGLLTCEATVNGHLYKTNYLTHRQTNTIIDVVLSPSHGIELSVGEKLVLNCTARTELNVGIDFNWEYPSSKHQHKKLVNRDLKTQSGSEMKKFLSTLTIDGVTRSDQGLYTCAASSGLMTKKNSTFVRVHEKGGGGSSPFIASVSDQHGVVYITENKNKTVVIPCLGSISNLNVSLVARYPEKRFVPDGNRISWDSKKGFTIPSYMISYAGMVFCEAKINDESYQSIMYIVVVVGYRIYDVVLSPSHGIELSVGEKLVLNCTARTELNVGIDFNWEYPSSKHQHKKLVNRDLKTQSGSEMKKFLSTLTIDGVTRSDQGLYTCAASSGLMTKKNSTFVRVHEKDKTHTCPPCPAPEAAGGPSVFLFPPKPKDTLMISRTPEVTCVVVDVSHEDPEVKFNWYVDGVEVHNAKTKPREEQYNSTYRVVSVLTVLHQDWLNGKEYKCKVSNKALPAPIEKTISKAKGQPREPQVYTLPPSREEMTKNQVSLTCLVKGFYPSDIAVEWESNGQPENNYKTTPPVLDSDGSFFLYSKLTVDKSRWQQGNVFSCSVMHEALHNHYTQKSLSLSPGK

SEQ ID NO: 9 - protein, 642 aa, synthetic construct
  source 1..642: note = PR1101 (R1D2-R2D3-linker-R2D2(M197Y)-R2D3-Fc)
SDTGRPFVEMYSEIPEIIHMTEGRELVIPCRVTSPNITVTLKKFPLDTLIPDGKRIIWDSRKGFIISNATYKEIGLLTCEATVNGHLYKTNYLTHRQTNTIIDVVLSPSHGIELSVGEKLVLNCTARTELNVGIDFNWEYPSSKHQHKKLVNRDLKTQSGSEMKKFLSTLTIDGVTRSDQGLYTCAASSGLMTKKNSTFVRVHEKGGGGSSPFIASVSDQHGVVYITENKNKTVVIPCLGSISNLNVSLCARYPEKRFVPDGNRISWDSKKGFTIPSYMISYAGYVFCEAKINDESYQSIMYIVVVVGYRIYDVVLSPSHGIELSVGEKLVLNCTARTELNVGIDFNWEYPSSKHQHKKLVNRDLKTQSGSEMKKFLSTLTIDGVTRSDQGLYTCAASSGLMTKKNSTFVRVHEKDKTHTCPPCPAPEAAGGPSVFLFPPKPKDTLMISRTPEVTCVVVDVSHEDPEVKFNWYVDGVEVHNAKTKPREEQYNSTYRVVSVLTVLHQDWLNGKEYKCKVSNKALPAPIEKTISKAKGQPREPQVYTLPPSREEMTKNQVSLTCLVKGFYPSDIAVEWESNGQPENNYKTTPPVLDSDGSFFLYSKLTVDKSRWQQGNVFSCSVMHEALHNHYTQKSLSLSPGK

SEQ ID NO: 10 - protein, 642 aa, synthetic construct
  source 1..642: note = PR1103 (R1D2-R2D3-linker-R2D2(F199Q)-R2D3-Fc)
SDTGRPFVEMYSEIPEIIHMTEGRELVIPCRVTSPNITVTLKKFPLDTLIPDGKRIIWDSRKGFIISNATYKEIGLLTCEATVNGHLYKTNYLTHRQTNTIIDVVLSPSHGIELSVGEKLVLNCTARTELNVGIDFNWEYPSSKHQHKKLVNRDLKTQSGSEMKKFLSTLTIDGVTRSDQGLYTCAASSGLMTKKNSTFVRVHEKGGGGSSPFIASVSDQHGVVYITENKNKTVVIPCLGSISNLNVSLCARYPEKRFVPDGNRISWDSKKGFTIPSYMISYAGMVQCEAKINDESYQSIMYIVVVVGYRIYDVVLSPSHGIELSVGEKLVLNCTARTELNVGIDFNWEYPSSKHQHKKLVNRDLKTQSGSEMKKFLSTLTIDGVTRSDQGLYTCAASSGLMTKKNSTFVRVHEKDKTHTCPPCPAPEAAGGPSVFLFPPKPKDTLMISRTPEVTCVVVDVSHEDPEVKFNWYVDGVEVHNAKTKPREEQYNSTYRVVSVLTVLHQDWLNGKEYKCKVSNKALPAPIEKTISKAKGQPREPQVYTLPPSREEMTKNQVSLTCLVKGFYPSDIAVEWESNGQPENNYKTTPPVLDSDGSFFLYSKLTVDKSRWQQGNVFSCSVMHEALHNHYTQKSLSLSPGK

SEQ ID NO: 11 - protein, 642 aa, synthetic construct
  source 1..642: note = PR1106 (R1D2-R2D3-linker-R2D2(M213N)-R2D3-Fc)
SDTGRPFVEMYSEIPEIIHMTEGRELVIPCRVTSPNITVTLKKFPLDTLIPDGKRIIWDSRKGFIISNATYKEIGLLTCEATVNGHLYKTNYLTHRQTNTIIDVVLSPSHGIELSVGEKLVLNCTARTELNVGIDFNWEYPSSKHQHKKLVNRDLKTQSGSEMKKFLSTLTIDGVTRSDQGLYTCAASSGLMTKKNSTFVRVHEKGGGGSSPFIASVSDQHGVVYITENKNKTVVIPCLGSISNLNVSLCARYPEKRFVPDGNRISWDSKKGFTIPSYMISYAGMVFCEAKINDESYQSINYIVVVVGYRIYDVVLSPSHGIELSVGEKLVLNCTARTELNVGIDFNWEYPSSKHQHKKLVNRDLKTQSGSEMKKFLSTLTIDGVTRSDQGLYTCAASSGLMTKKNSTFVRVHEKDKTHTCPPCPAPEAAGGPSVFLFPPKPKDTLMISRTPEVTCVVVDVSHEDPEVKFNWYVDGVEVHNAKTKPREEQYNSTYRVVSVLTVLHQDWLNGKEYKCKVSNKALPAPIEKTISKAKGQPREPQVYTLPPSREEMTKNQVSLTCLVKGFYPSDIAVEWESNGQPENNYKTTPPVLDSDGSFFLYSKLTVDKSRWQQGNVFSCSVMHEALHNHYTQKSLSLSPGK

SEQ ID NO: 12 - protein, 642 aa, synthetic construct
  source 1..642: note = PR1107 (R1D2-R2D3-linker-R2D2(I215F)-R2D3-Fc)
SDTGRPFVEMYSEIPEIIHMTEGRELVIPCRVTSPNITVTLKKFPLDTLIPDGKRIIWDSRKGFIISNATYKEIGLLTCEATVNGHLYKTNYLTHRQTNTIIDVVLSPSHGIELSVGEKLVLNCTARTELNVGIDFNWEYPSSKHQHKKLVNRDLKTQSGSEMKKFLSTLTIDGVTRSDQGLYTCAASSGLMTKKNSTFVRVHEKGGGGSSPFIASVSDQHGVVYITENKNKTVVIPCLGSISNLNVSLCARYPEKRFVPDGNRISWDSKKGFTIPSYMISYAGMVFCEAKINDESYQSIMYFVVVVGYRIYDVVLSPSHGIELSVGEKLVLNCTARTELNVGIDFNWEYPSSKHQHKKLVNRDLKTQSGSEMKKFLSTLTIDGVTRSDQGLYTCAASSGLMTKKNSTFVRVHEKDKTHTCPPCPAPEAAGGPSVFLFPPKPKDTLMISRTPEVTCVVVDVSHEDPEVKFNWYVDGVEVHNAKTKPREEQYNSTYRVVSVLTVLHQDWLNGKEYKCKVSNKALPAPIEKTISKAKGQPREPQVYTLPPSREEMTKNQVSLTCLVKGFYPSDIAVEWESNGQPENNYKTTPPVLDSDGSFFLYSKLTVDKSRWQQGNVFSCSVMHEALHNHYTQKSLSLSPGK

SEQ ID NO: 13 - protein, 642 aa, synthetic construct
  source 1..642: note = PR1108 (R1D2-R2D3-linker-R2D2(I215H)-R2D3-Fc)
SDTGRPFVEMYSEIPEIIHMTEGRELVIPCRVTSPNITVTLKKFPLDTLIPDGKRIIWDSRKGFIISNATYKEIGLLTCEATVNGHLYKTNYLTHRQTNTIIDVVLSPSHGIELSVGEKLVLNCTARTELNVGIDFNWEYPSSKHQHKKLVNRDLKTQSGSEMKKFLSTLTIDGVTRSDQGLYTCAASSGLMTKKNSTFVRVHEKGGGGSSPFIASVSDQHGVVYITENKNKTVVIPCLGSISNLNVSLCARYPEKRFVPDGNRISWDSKKGFTIPSYMISYAGMVFCEAKINDESYQSIMYHVVVVGYRIYDVVLSPSHGIELSVGEKLVLNCTARTELNVGIDFNWEYPSSKHQHKKLVNRDLKTQSGSEMKKFLSTLTIDGVTRSDQGLYTCAASSGLMTKKNSTFVRVHEKDKTHTCPPCPAPEAAGGPSVFLFPPKPKDTLMISRTPEVTCVVVDVSHEDPEVKFNWYVDGVEVHNAKTKPREEQYNSTYRVVSVLTVLHQDWLNGKEYKCKVSNKALPAPIEKTISKAKGQPREPQVYTLPPSREEMTKNQVSLTCLVKGFYPSDIAVEWESNGQPENNYKTTPPVLDSDGSFFLYSKLTVDKSRWQQGNVFSCSVMHEALHNHYTQKSLSLSPGK

SEQ ID NO: 14 - protein, 642 aa, synthetic construct
  source 1..642: note = PR1109 (R1D2-R2D3-linker-R2D2(V219I)-R2D3-Fc)
SDTGRPFVEMYSEIPEIIHMTEGRELVIPCRVTSPNITVTLKKFPLDTLIPDGKRIIWDSRKGFIISNATYKEIGLLTCEATVNGHLYKTNYLTHRQTNTIIDVVLSPSHGIELSVGEKLVLNCTARTELNVGIDFNWEYPSSKHQHKKLVNRDLKTQSGSEMKKFLSTLTIDGVTRSDQGLYTCAASSGLMTKKNSTFVRVHEKGGGGSSPFIASVSDQHGVVYITENKNKTVVIPCLGSISNLNVSLCARYPEKRFVPDGNRISWDSKKGFTIPSYMISYAGMVFCEAKINDESYQSIMYIVVVIGYRIYDVVLSPSHGIELSVGEKLVLNCTARTELNVGIDFNWEYPSSKHQHKKLVNRDLKTQSGSEMKKFLSTLTIDGVTRSDQGLYTCAASSGLMTKKNSTFVRVHEKDKTHTCPPCPAPEAAGGPSVFLFPPKPKDTLMISRTPEVTCVVVDVSHEDPEVKFNWYVDGVEVHNAKTKPREEQYNSTYRVVSVLTVLHQDWLNGKEYKCKVSNKALPAPIEKTISKAKGQPREPQVYTLPPSREEMTKNQVSLTCLVKGFYPSDIAVEWESNGQPENNYKTTPPVLDSDGSFFLYSKLTVDKSRWQQGNVFSCSVMHEALHNHYTQKSLSLSPGK

SEQ ID NO: 15 - protein, 642 aa, synthetic construct
  source 1..642: note = PR1110 (R1D2-R2D3-linker-R2D2(Y221N)-R2D3-Fc)
SDTGRPFVEMYSEIPEIIHMTEGRELVIPCRVTSPNITVTLKKFPLDTLIPDGKRIIWDSRKGFIISNATYKEIGLLTCEATVNGHLYKTNYLTHRQTNTIIDVVLSPSHGIELSVGEKLVLNCTARTELNVGIDFNWEYPSSKHQHKKLVNRDLKTQSGSEMKKFLSTLTIDGVTRSDQGLYTCAASSGLMTKKNSTFVRVHEKGGGGSSPFIASVSDQHGVVYITENKNKTVVIPCLGSISNLNVSLCARYPEKRFVPDGNRISWDSKKGFTIPSYMISYAGMVFCEAKINDESYQSIMYIVVVVGNRIYDVVLSPSHGIELSVGEKLVLNCTARTELNVGIDFNWEYPSSKHQHKKLVNRDLKTQSGSEMKKFLSTLTIDGVTRSDQGLYTCAASSGLMTKKNSTFVRVHEKDKTHTCPPCPAPEAAGGPSVFLFPPKPKDTLMISRTPEVTCVVVDVSHEDPEVKFNWYVDGVEVHNAKTKPREEQYNSTYRVVSVLTVLHQDWLNGKEYKCKVSNKALPAPIEKTISKAKGQPREPQVYTLPPSREEMTKNQVSLTCLVKGFYPSDIAVEWESNGQPENNYKTTPPVLDSDGSFFLYSKLTVDKSRWQQGNVFSCSVMHEALHNHYTQKSLSLSPGK

SEQ ID NO: 16 - protein, 642 aa, synthetic construct
  source 1..642: note = PR1111 (R1D2-R2D3-linker-R2D2-R2D3(D257Q)-Fc)
SDTGRPFVEMYSEIPEIIHMTEGRELVIPCRVTSPNITVTLKKFPLDTLIPDGKRIIWDSRKGFIISNATYKEIGLLTCEATVNGHLYKTNYLTHRQTNTIIDVVLSPSHGIELSVGEKLVLNCTARTELNVGIDFNWEYPSSKHQHKKLVNRDLKTQSGSEMKKFLSTLTIDGVTRSDQGLYTCAASSGLMTKKNSTFVRVHEKGGGGSSPFIASVSDQHGVVYITENKNKTVVIPCLGSISNLNVSLCARYPEKRFVPDGNRISWDSKKGFTIPSYMISYAGMVFCEAKINDESYQSIMYIVVVVGYRIYDVVLSPSHGIELSVGEKLVLNCTARTELNVGIQFNWEYPSSKHQHKKLVNRDLKTQSGSEMKKFLSTLTIDGVTRSDQGLYTCAASSGLMTKKNSTFVRVHEKDKTHTCPPCPAPEAAGGPSVFLFPPKPKDTLMISRTPEVTCVVVDVSHEDPEVKFNWYVDGVEVHNAKTKPREEQYNSTYRVVSVLTVLHQDWLNGKEYKCKVSNKALPAPIEKTISKAKGQPREPQVYTLPPSREEMTKNQVSLTCLVKGFYPSDIAVEWESNGQPENNYKTTPPVLDSDGSFFLYSKLTVDKSRWQQGNVFSCSVMHEALHNHYTQKSLSLSPGK

SEQ ID NO: 17 - protein, 642 aa, synthetic construct
  source 1..642: note = PR1112 (R1D2-R2D3-linker-R2D2-R2D3(D257T)-Fc)
SDTGRPFVEMYSEIPEIIHMTEGRELVIPCRVTSPNITVTLKKFPLDTLIPDGKRIIWDSRKGFIISNATYKEIGLLTCEATVNGHLYKTNYLTHRQTNTIIDVVLSPSHGIELSVGEKLVLNCTARTELNVGIDFNWEYPSSKHQHKKLVNRDLKTQSGSEMKKFLSTLTIDGVTRSDQGLYTCAASSGLMTKKNSTFVRVHEKGGGGSSPFIASVSDQHGVVYITENKNKTVVIPCLGSISNLNVSLCARYPEKRFVPDGNRISWDSKKGFTIPSYMISYAGMVFCEAKINDESYQSIMYIVVVVGYRIYDVVLSPSHGIELSVGEKLVLNCTARTELNVGITFNWEYPSSKHQHKKLVNRDLKTQSGSEMKKFLSTLTIDGVTRSDQGLYTCAASSGLMTKKNSTFVRVHEKDKTHTCPPCPAPEAAGGPSVFLFPPKPKDTLMISRTPEVTCVVVDVSHEDPEVKFNWYVDGVEVHNAKTKPREEQYNSTYRVVSVLTVLHQDWLNGKEYKCKVSNKALPAPIEKTISKAKGQPREPQVYTLPPSREEMTKNQVSLTCLVKGFYPSDIAVEWESNGQPENNYKTTPPVLDSDGSFFLYSKLTVDKSRWQQGNVFSCSVMHEALHNHYTQKSLSLSPGK

SEQ ID NO: 18 - protein, 642 aa, synthetic construct
  source 1..642: note = PR1113 (R1D2-R2D3-linker-R2D2-R2D3(N274F)-Fc)
SDTGRPFVEMYSEIPEIIHMTEGRELVIPCRVTSPNITVTLKKFPLDTLIPDGKRIIWDSRKGFIISNATYKEIGLLTCEATVNGHLYKTNYLTHRQTNTIIDVVLSPSHGIELSVGEKLVLNCTARTELNVGIDFNWEYPSSKHQHKKLVNRDLKTQSGSEMKKFLSTLTIDGVTRSDQGLYTCAASSGLMTKKNSTFVRVHEKGGGGSSPFIASVSDQHGVVYITENKNKTVVIPCLGSISNLNVSLCARYPEKRFVPDGNRISWDSKKGFTIPSYMISYAGMVFCEAKINDESYQSIMYIVVVVGYRIYDVVLSPSHGIELSVGEKLVLNCTARTELNVGIDFNWEYPSSKHQHKKLVFRDLKTQSGSEMKKFLSTLTIDGVTRSDQGLYTCAASSGLMTKKNSTFVRVHEKDKTHTCPPCPAPEAAGGPSVFLFPPKPKDTLMISRTPEVTCVVVDVSHEDPEVKFNWYVDGVEVHNAKTKPREEQYNSTYRVVSVLTVLHQDWLNGKEYKCKVSNKALPAPIEKTISKAKGQPREPQVYTLPPSREEMTKNQVSLTCLVKGFYPSDIAVEWESNGQPENNYKTTPPVLDSDGSFFLYSKLTVDKSRWQQGNVFSCSVMHEALHNHYTQKSLSLSPGK

SEQ ID NO: 19 - protein, 642 aa, synthetic construct
  source 1..642: note = PR1114 (R1D2-R2D3-linker-R2D2-R2D3(N274I)-Fc)
SDTGRPFVEMYSEIPEIIHMTEGRELVIPCRVTSPNITVTLKKFPLDTLIPDGKRIIWDSRKGFIISNATYKEIGLLTCEATVNGHLYKTNYLTHRQTNTIIDVVLSPSHGIELSVGEKLVLNCTARTELNVGIDFNWEYPSSKHQHKKLVNRDLKTQSGSEMKKFLSTLTIDGVTRSDQGLYTCAASSGLMTKKNSTFVRVHEKGGGGSSPFIASVSDQHGVVYITENKNKTVVIPCLGSISNLNVSLCARYPEKRFVPDGNRISWDSKKGFTIPSYMISYAGMVFCEAKINDESYQSIMYIVVVVGYRIYDVVLSPSHGIELSVGEKLVLNCTARTELNVGIDFNWEYPSSKHQHKKLVIRDLKTQSGSEMKKFLSTLTIDGVTRSDQGLYTCAASSGLMTKKNSTFVRVHEKDKTHTCPPCPAPEAAGGPSVFLFPPKPKDTLMISRTPEVTCVVVDVSHEDPEVKFNWYVDGVEVHNAKTKPREEQYNSTYRVVSVLTVLHQDWLNGKEYKCKVSNKALPAPIEKTISKAKGQPREPQVYTLPPSREEMTKNQVSLTCLVKGFYPSDIAVEWESNGQPENNYKTTPPVLDSDGSFFLYSKLTVDKSRWQQGNVFSCSVMHEALHNHYTQKSLSLSPGK

SEQ ID NO: 20 - protein, 642 aa, synthetic construct
  source 1..642: note = PR1115 (R1D2-R2D3-linker-R2D2-R2D3(R257L)-Fc)
SDTGRPFVEMYSEIPEIIHMTEGRELVIPCRVTSPNITVTLKKFPLDTLIPDGKRIIWDSRKGFIISNATYKEIGLLTCEATVNGHLYKTNYLTHRQTNTIIDVVLSPSHGIELSVGEKLVLNCTARTELNVGIDFNWEYPSSKHQHKKLVNRDLKTQSGSEMKKFLSTLTIDGVTRSDQGLYTCAASSGLMTKKNSTFVRVHEKGGGGSSPFIASVSDQHGVVYITENKNKTVVIPCLGSISNLNVSLCARYPEKRFVPDGNRISWDSKKGFTIPSYMISYAGMVFCEAKINDESYQSIMYIVVVVGYRIYDVVLSPSHGIELSVGEKLVLNCTARTELNVGIDFNWEYPSSKHQHKKLVNLDLKTQSGSEMKKFLSTLTIDGVTRSDQGLYTCAASSGLMTKKNSTFVRVHEKDKTHTCPPCPAPEAAGGPSVFLFPPKPKDTLMISRTPEVTCVVVDVSHEDPEVKFNWYVDGVEVHNAKTKPREEQYNSTYRVVSVLTVLHQDWLNGKEYKCKVSNKALPAPIEKTISKAKGQPREPQVYTLPPSREEMTKNQVSLTCLVKGFYPSDIAVEWESNGQPENNYKTTPPVLDSDGSFFLYSKLTVDKSRWQQGNVFSCSVMHEALHNHYTQKSLSLSPGK

SEQ ID NO: 21 - protein, 642 aa, synthetic construct
  source 1..642: note = PR1116 (R1D2-R2D3-linker-R2D2-R2D3(R257E)-Fc)
SDTGRPFVEMYSEIPEIIHMTEGRELVIPCRVTSPNITVTLKKFPLDTLIPDGKRIIWDSRKGFIISNATYKEIGLLTCEATVNGHLYKTNYLTHRQTNTIIDVVLSPSHGIELSVGEKLVLNCTARTELNVGIDFNWEYPSSKHQHKKLVNRDLKTQSGSEMKKFLSTLTIDGVTRSDQGLYTCAASSGLMTKKNSTFVRVHEKGGGGSSPFIASVSDQHGVVYITENKNKTVVIPCLGSISNLNVSLCARYPEKRFVPDGNRISWDSKKGFTIPSYMISYAGMVFCEAKINDESYQSIMYIVVVVGYRIYDVVLSPSHGIELSVGEKLVLNCTARTELNVGIDFNWEYPSSKHQHKKLVNEDLKTQSGSEMKKFLSTLTIDGVTRSDQGLYTCAASSGLMTKKNSTFVRVHEKDKTHTCPPCPAPEAAGGPSVFLFPPKPKDTLMISRTPEVTCVVVDVSHEDPEVKFNWYVDGVEVHNAKTKPREEQYNSTYRVVSVLTVLHQDWLNGKEYKCKVSNKALPAPIEKTISKAKGQPREPQVYTLPPSREEMTKNQVSLTCLVKGFYPSDIAVEWESNGQPENNYKTTPPVLDSDGSFFLYSKLTVDKSRWQQGNVFSCSVMHEALHNHYTQKSLSLSPGK

SEQ ID NO: 22 - protein, 642 aa, synthetic construct
  source 1..642: note = PR1118 (R1D2-R2D3-linker-R2D2-R2D3(D276Q)-Fc)
SDTGRPFVEMYSEIPEIIHMTEGRELVIPCRVTSPNITVTLKKFPLDTLIPDGKRIIWDSRKGFIISNATYKEIGLLTCEATVNGHLYKTNYLTHRQTNTIIDVVLSPSHGIELSVGEKLVLNCTARTELNVGIDFNWEYPSSKHQHKKLVNRDLKTQSGSEMKKFLSTLTIDGVTRSDQGLYTCAASSGLMTKKNSTFVRVHEKGGGGSSPFIASVSDQHGVVYITENKNKTVVIPCLGSISNLNVSLCARYPEKRFVPDGNRISWDSKKGFTIPSYMISYAGMVFCEAKINDESYQSIMYIVVVVGYRIYDVVLSPSHGIELSVGEKLVLNCTARTELNVGIDFNWEYPSSKHQHKKLVNRQLKTQSGSEMKKFLSTLTIDGVTRSDQGLYTCAASSGLMTKKNSTFVRVHEKDKTHTCPPCPAPEAAGGPSVFLFPPKPKDTLMISRTPEVTCVVVDVSHEDPEVKFNWYVDGVEVHNAKTKPREEQYNSTYRVVSVLTVLHQDWLNGKEYKCKVSNKALPAPIEKTISKAKGQPREPQVYTLPPSREEMTKNQVSLTCLVKGFYPSDIAVEWESNGQPENNYKTTPPVLDSDGSFFLYSKLTVDKSRWQQGNVFSCSVMHEALHNHYTQKSLSLSPGK

SEQ ID NO: 23 - protein, 642 aa, synthetic construct
  source 1..642: note = PR1119 (R1D2-R2D3-linker-R2D2-R2D3(L277R)-Fc)
SDTGRPFVEMYSEIPEIIHMTEGRELVIPCRVTSPNITVTLKKFPLDTLIPDGKRIIWDSRKGFIISNATYKEIGLLTCEATVNGHLYKTNYLTHRQTNTIIDVVLSPSHGIELSVGEKLVLNCTARTELNVGIDFNWEYPSSKHQHKKLVNRDLKTQSGSEMKKFLSTLTIDGVTRSDQGLYTCAASSGLMTKKNSTFVRVHEKGGGGSSPFIASVSDQHGVVYITENKNKTVVIPCLGSISNLNVSLCARYPEKRFVPDGNRISWDSKKGFTIPSYMISYAGMVFCEAKINDESYQSIMYIVVVVGYRIYDVVLSPSHGIELSVGEKLVLNCTARTELNVGIDFNWEYPSSKHQHKKLVNRDRKTQSGSEMKKFLSTLTIDGVTRSDQGLYTCAASSGLMTKKNSTFVRVHEKDKTHTCPPCPAPEAAGGPSVFLFPPKPKDTLMISRTPEVTCVVVDVSHEDPEVKFNWYVDGVEVHNAKTKPREEQYNSTYRVVSVLTVLHQDWLNGKEYKCKVSNKALPAPIEKTISKAKGQPREPQVYTLPPSREEMTKNQVSLTCLVKGFYPSDIAVEWESNGQPENNYKTTPPVLDSDGSFFLYSKLTVDKSRWQQGNVFSCSVMHEALHNHYTQKSLSLSPGK

SEQ ID NO: 24 - protein, 642 aa, synthetic construct
  source 1..642: note = PR1120 (R1D2-R2D3-linker-R2D2-R2D3(K278D)-Fc)
SDTGRPFVEMYSEIPEIIHMTEGRELVIPCRVTSPNITVTLKKFPLDTLIPDGKRIIWDSRKGFIISNATYKEIGLLTCEATVNGHLYKTNYLTHRQTNTIIDVVLSPSHGIELSVGEKLVLNCTARTELNVGIDFNWEYPSSKHQHKKLVNRDLKTQSGSEMKKFLSTLTIDGVTRSDQGLYTCAASSGLMTKKNSTFVRVHEKGGGGSSPFIASVSDQHGVVYITENKNKTVVIPCLGSISNLNVSLCARYPEKRFVPDGNRISWDSKKGFTIPSYMISYAGMVFCEAKINDESYQSIMYIVVVVGYRIYDVVLSPSHGIELSVGEKLVLNCTARTELNVGIDFNWEYPSSKHQHKKLVNRDLDTQSGSEMKKFLSTLTIDGVTRSDQGLYTCAASSGLMTKKNSTFVRVHEKDKTHTCPPCPAPEAAGGPSVFLFPPKPKDTLMISRTPEVTCVVVDVSHEDPEVKFNWYVDGVEVHNAKTKPREEQYNSTYRVVSVLTVLHQDWLNGKEYKCKVSNKALPAPIEKTISKAKGQPREPQVYTLPPSREEMTKNQVSLTCLVKGFYPSDIAVEWESNGQPENNYKTTPPVLDSDGSFFLYSKLTVDKSRWQQGNVFSCSVMHEALHNHYTQKSLSLSPGK

SEQ ID NO: 25 - protein, 642 aa, synthetic construct
  source 1..642: note = PR1121 (R1D2-R2D3-linker-R2D2-R2D3(K278S)-Fc)
SDTGRPFVEMYSEIPEIIHMTEGRELVIPCRVTSPNITVTLKKFPLDTLIPDGKRIIWDSRKGFIISNATYKEIGLLTCEATVNGHLYKTNYLTHRQTNTIIDVVLSPSHGIELSVGEKLVLNCTARTELNVGIDFNWEYPSSKHQHKKLVNRDLKTQSGSEMKKFLSTLTIDGVTRSDQGLYTCAASSGLMTKKNSTFVRVHEKGGGGSSPFIASVSDQHGVVYITENKNKTVVIPCLGSISNLNVSLCARYPEKRFVPDGNRISWDSKKGFTIPSYMISYAGMVFCEAKINDESYQSIMYIVVVVGYRIYDVVLSPSHGIELSVGEKLVLNCTARTELNVGIDFNWEYPSSKHQHKKLVNRDLSTQSGSEMKKFLSTLTIDGVTRSDQGLYTCAASSGLMTKKNSTFVRVHEKDKTHTCPPCPAPEAAGGPSVFLFPPKPKDTLMISRTPEVTCVVVDVSHEDPEVKFNWYVDGVEVHNAKTKPREEQYNSTYRVVSVLTVLHQDWLNGKEYKCKVSNKALPAPIEKTISKAKGQPREPQVYTLPPSREEMTKNQVSLTCLVKGFYPSDIAVEWESNGQPENNYKTTPPVLDSDGSFFLYSKLTVDKSRWQQGNVFSCSVMHEALHNHYTQKSLSLSPGK

SEQ ID NO: 26 - protein, 642 aa, synthetic construct
  source 1..642: note = PR1122 (R1D2-R2D3-linker-R2D2-R2D3(K278E)-Fc)
SDTGRPFVEMYSEIPEIIHMTEGRELVIPCRVTSPNITVTLKKFPLDTLIPDGKRIIWDSRKGFIISNATYKEIGLLTCEATVNGHLYKTNYLTHRQTNTIIDVVLSPSHGIELSVGEKLVLNCTARTELNVGIDFNWEYPSSKHQHKKLVNRDLKTQSGSEMKKFLSTLTIDGVTRSDQGLYTCAASSGLMTKKNSTFVRVHEKGGGGSSPFIASVSDQHGVVYITENKNKTVVIPCLGSISNLNVSLCARYPEKRFVPDGNRISWDSKKGFTIPSYMISYAGMVFCEAKINDESYQSIMYIVVVVGYRIYDVVLSPSHGIELSVGEKLVLNCTARTELNVGIDFNWEYPSSKHQHKKLVNRDLETQSGSEMKKFLSTLTIDGVTRSDQGLYTCAASSGLMTKKNSTFVRVHEKDKTHTCPPCPAPEAAGGPSVFLFPPKPKDTLMISRTPEVTCVVVDVSHEDPEVKFNWYVDGVEVHNAKTKPREEQYNSTYRVVSVLTVLHQDWLNGKEYKCKVSNKALPAPIEKTISKAKGQPREPQVYTLPPSREEMTKNQVSLTCLVKGFYPSDIAVEWESNGQPENNYKTTPPVLDSDGSFFLYSKLTVDKSRWQQGNVFSCSVMHEALHNHYTQKSLSLSPGK

SEQ ID NO: 27 - protein, 642 aa, synthetic construct
  source 1..642: note = PR1123 (R1D2-R2D3-linker-R2D2-R2D3(Q280E)-Fc)
SDTGRPFVEMYSEIPEIIHMTEGRELVIPCRVTSPNITVTLKKFPLDTLIPDGKRIIWDSRKGFIISNATYKEIGLLTCEATVNGHLYKTNYLTHRQTNTIIDVVLSPSHGIELSVGEKLVLNCTARTELNVGIDFNWEYPSSKHQHKKLVNRDLKTQSGSEMKKFLSTLTIDGVTRSDQGLYTCAASSGLMTKKNSTFVRVHEKGGGGSSPFIASVSDQHGVVYITENKNKTVVIPCLGSISNLNVSLCARYPEKRFVPDGNRISWDSKKGFTIPSYMISYAGMVFCEAKINDESYQSIMYIVVVVGYRIYDVVLSPSHGIELSVGEKLVLNCTARTELNVGIDFNWEYPSSKHQHKKLVNRDLKTESGSEMKKFLSTLTIDGVTRSDQGLYTCAASSGLMTKKNSTFVRVHEKDKTHTCPPCPAPEAAGGPSVFLFPPKPKDTLMISRTPEVTCVVVDVSHEDPEVKFNWYVDGVEVHNAKTKPREEQYNSTYRVVSVLTVLHQDWLNGKEYKCKVSNKALPAPIEKTISKAKGQPREPQVYTLPPSREEMTKNQVSLTCLVKGFYPSDIAVEWESNGQPENNYKTTPPVLDSDGSFFLYSKLTVDKSRWQQGNVFSCSVMHEALHNHYTQKSLSLSPGK

SEQ ID NO: 28 - protein, 642 aa, synthetic construct
  source 1..642: note = PR1124 (R1D2-R2D3-linker-R2D2-R2D3(S283T)-Fc)
SDTGRPFVEMYSEIPEIIHMTEGRELVIPCRVTSPNITVTLKKFPLDTLIPDGKRIIWDSRKGFIISNATYKEIGLLTCEATVNGHLYKTNYLTHRQTNTIIDVVLSPSHGIELSVGEKLVLNCTARTELNVGIDFNWEYPSSKHQHKKLVNRDLKTQSGSEMKKFLSTLTIDGVTRSDQGLYTCAASSGLMTKKNSTFVRVHEKGGGGSSPFIASVSDQHGVVYITENKNKTVVIPCLGSISNLNVSLCARYPEKRFVPDGNRISWDSKKGFTIPSYMISYAGMVFCEAKINDESYQSIMYIVVVVGYRIYDVVLSPSHGIELSVGEKLVLNCTARTELNVGIDFNWEYPSSKHQHKKLVNRDLKTQSGTEMKKFLSTLTIDGVTRSDQGLYTCAASSGLMTKKNSTFVRVHEKDKTHTCPPCPAPEAAGGPSVFLFPPKPKDTLMISRTPEVTCVVVDVSHEDPEVKFNWYVDGVEVHNAKTKPREEQYNSTYRVVSVLTVLHQDWLNGKEYKCKVSNKALPAPIEKTISKAKGQPREPQVYTLPPSREEMTKNQVSLTCLVKGFYPSDIAVEWESNGQPENNYKTTPPVLDSDGSFFLYSKLTVDKSRWQQGNVFSCSVMHEALHNHYTQKSLSLSPGK

SEQ ID NO: 29 - protein, 642 aa, synthetic construct
  source 1..642: note = PR1125 (R1D2-R2D3-linker-R2D2-R2D3(E284H)-Fc)
SDTGRPFVEMYSEIPEIIHMTEGRELVIPCRVTSPNITVTLKKFPLDTLIPDGKRIIWDSRKGFIISNATYKEIGLLTCEATVNGHLYKTNYLTHRQTNTIIDVVLSPSHGIELSVGEKLVLNCTARTELNVGIDFNWEYPSSKHQHKKLVNRDLKTQSGSEMKKFLSTLTIDGVTRSDQGLYTCAASSGLMTKKNSTFVRVHEKGGGGSSPFIASVSDQHGVVYITENKNKTVVIPCLGSISNLNVSLCARYPEKRFVPDGNRISWDSKKGFTIPSYMISYAGMVFCEAKINDESYQSIMYIVVVVGYRIYDVVLSPSHGIELSVGEKLVLNCTARTELNVGIDFNWEYPSSKHQHKKLVNRDLKTQSGSHMKKFLSTLTIDGVTRSDQGLYTCAASSGLMTKKNSTFVRVHEKDKTHTCPPCPAPEAAGGPSVFLFPPKPKDTLMISRTPEVTCVVVDVSHEDPEVKFNWYVDGVEVHNAKTKPREEQYNSTYRVVSVLTVLHQDWLNGKEYKCKVSNKALPAPIEKTISKAKGQPREPQVYTLPPSREEMTKNQVSLTCLVKGFYPSDIAVEWESNGQPENNYKTTPPVLDSDGSFFLYSKLTVDKSRWQQGNVFSCSVMHEALHNHYTQKSLSLSPGK

SEQ ID NO: 30 - protein, 642 aa, synthetic construct
  source 1..642: note = PR1126 (R1D2-R2D3-linker-R2D2-R2D3(F288Y)-Fc)
SDTGRPFVEMYSEIPEIIHMTEGRELVIPCRVTSPNITVTLKKFPLDTLIPDGKRIIWDSRKGFIISNATYKEIGLLTCEATVNGHLYKTNYLTHRQTNTIIDVVLSPSHGIELSVGEKLVLNCTARTELNVGIDFNWEYPSSKHQHKKLVNRDLKTQSGSEMKKFLSTLTIDGVTRSDQGLYTCAASSGLMTKKNSTFVRVHEKGGGGSSPFIASVSDQHGVVYITENKNKTVVIPCLGSISNLNVSLCARYPEKRFVPDGNRISWDSKKGFTIPSYMISYAGMVFCEAKINDESYQSIMYIVVVVGYRIYDVVLSPSHGIELSVGEKLVLNCTARTELNVGIDFNWEYPSSKHQHKKLVNRDLKTQSGSEMKKYLSTLTIDGVTRSDQGLYTCAASSGLMTKKNSTFVRVHEKDKTHTCPPCPAPEAAGGPSVFLFPPKPKDTLMISRTPEVTCVVVDVSHEDPEVKFNWYVDGVEVHNAKTKPREEQYNSTYRVVSVLTVLHQDWLNGKEYKCKVSNKALPAPIEKTISKAKGQPREPQVYTLPPSREEMTKNQVSLTCLVKGFYPSDIAVEWESNGQPENNYKTTPPVLDSDGSFFLYSKLTVDKSRWQQGNVFSCSVMHEALHNHYTQKSLSLSPGK

SEQ ID NO: 31 - protein, 642 aa, synthetic construct
  source 1..642: note = PR1127 (R1D2-R2D3-linker-R2D2-R2D3(L289Y)-Fc)
SDTGRPFVEMYSEIPEIIHMTEGRELVIPCRVTSPNITVTLKKFPLDTLIPDGKRIIWDSRKGFIISNATYKEIGLLTCEATVNGHLYKTNYLTHRQTNTIIDVVLSPSHGIELSVGEKLVLNCTARTELNVGIDFNWEYPSSKHQHKKLVNRDLKTQSGSEMKKFLSTLTIDGVTRSDQGLYTCAASSGLMTKKNSTFVRVHEKGGGGSSPFIASVSDQHGVVYITENKNKTVVIPCLGSISNLNVSLCARYPEKRFVPDGNRISWDSKKGFTIPSYMISYAGMVFCEAKINDESYQSIMYIVVVVGYRIYDVVLSPSHGIELSVGEKLVLNCTARTELNVGIDFNWEYPSSKHQHKKLVNRDLKTQSGSEMKKFYSTLTIDGVTRSDQGLYTCAASSGLMTKKNSTFVRVHEKDKTHTCPPCPAPEAAGGPSVFLFPPKPKDTLMISRTPEVTCVVVDVSHEDPEVKFNWYVDGVEVHNAKTKPREEQYNSTYRVVSVLTVLHQDWLNGKEYKCKVSNKALPAPIEKTISKAKGQPREPQVYTLPPSREEMTKNQVSLTCLVKGFYPSDIAVEWESNGQPENNYKTTPPVLDSDGSFFLYSKLTVDKSRWQQGNVFSCSVMHEALHNHYTQKSLSLSPGK

SEQ ID NO: 32 - protein, 642 aa, synthetic construct
  source 1..642: note = PR1128 (R1D2-R2D3-linker-R2D2-R2D3(L313Y)-Fc)
SDTGRPFVEMYSEIPEIIHMTEGRELVIPCRVTSPNITVTLKKFPLDTLIPDGKRIIWDSRKGFIISNATYKEIGLLTCEATVNGHLYKTNYLTHRQTNTIIDVVLSPSHGIELSVGEKLVLNCTARTELNVGIDFNWEYPSSKHQHKKLVNRDLKTQSGSEMKKFLSTLTIDGVTRSDQGLYTCAASSGLMTKKNSTFVRVHEKGGGGSSPFIASVSDQHGVVYITENKNKTVVIPCLGSISNLNVSLCARYPEKRFVPDGNRISWDSKKGFTIPSYMISYAGMVFCEAKINDESYQSIMYIVVVVGYRIYDVVLSPSHGIELSVGEKLVLNCTARTELNVGIDFNWEYPSSKHQHKKLVNRDLKTQSGSEMKKFLSTLTIDGVTRSDQGLYTCAASSGYMTKKNSTFVRVHEKDKTHTCPPCPAPEAAGGPSVFLFPPKPKDTLMISRTPEVTCVVVDVSHEDPEVKFNWYVDGVEVHNAKTKPREEQYNSTYRVVSVLTVLHQDWLNGKEYKCKVSNKALPAPIEKTISKAKGQPREPQVYTLPPSREEMTKNQVSLTCLVKGFYPSDIAVEWESNGQPENNYKTTPPVLDSDGSFFLYSKLTVDKSRWQQGNVFSCSVMHEALHNHYTQKSLSLSPGK

SEQ ID NO: 33 - protein, 642 aa, synthetic construct
  source 1..642: note = PR1129 (R1D2-R2D3-linker-R2D2-R2D3(M314S)-Fc)
SDTGRPFVEMYSEIPEIIHMTEGRELVIPCRVTSPNITVTLKKFPLDTLIPDGKRIIWDSRKGFIISNATYKEIGLLTCEATVNGHLYKTNYLTHRQTNTIIDVVLSPSHGIELSVGEKLVLNCTARTELNVGIDFNWEYPSSKHQHKKLVNRDLKTQSGSEMKKFLSTLTIDGVTRSDQGLYTCAASSGLMTKKNSTFVRVHEKGGGGSSPFIASVSDQHGVVYITENKNKTVVIPCLGSISNLNVSLCARYPEKRFVPDGNRISWDSKKGFTIPSYMISYAGMVFCEAKINDESYQSIMYIVVVVGYRIYDVVLSPSHGIELSVGEKLVLNCTARTELNVGIDFNWEYPSSKHQHKKLVNRDLKTQSGSEMKKFLSTLTIDGVTRSDQGLYTCAASSGLSTKKNSTFVRVHEKDKTHTCPPCPAPEAAGGPSVFLFPPKPKDTLMISRTPEVTCVVVDVSHEDPEVKFNWYVDGVEVHNAKTKPREEQYNSTYRVVSVLTVLHQDWLNGKEYKCKVSNKALPAPIEKTISKAKGQPREPQVYTLPPSREEMTKNQVSLTCLVKGFYPSDIAVEWESNGQPENNYKTTPPVLDSDGSFFLYSKLTVDKSRWQQGNVFSCSVMHEALHNHYTQKSLSLSPGK

SEQ ID NO: 34 - protein, 642 aa, synthetic construct
  source 1..642: note = PR1130 (R1D2-R2D3-linker-R2D2-R2D3(M314Q)-Fc)
SDTGRPFVEMYSEIPEIIHMTEGRELVIPCRVTSPNITVTLKKFPLDTLIPDGKRIIWDSRKGFIISNATYKEIGLLTCEATVNGHLYKTNYLTHRQTNTIIDVVLSPSHGIELSVGEKLVLNCTARTELNVGIDFNWEYPSSKHQHKKLVNRDLKTQSGSEMKKFLSTLTIDGVTRSDQGLYTCAASSGLMTKKNSTFVRVHEKGGGGSSPFIASVSDQHGVVYITENKNKTVVIPCLGSISNLNVSLCARYPEKRFVPDGNRISWDSKKGFTIPSYMISYAGMVFCEAKINDESYQSIMYIVVVVGYRIYDVVLSPSHGIELSVGEKLVLNCTARTELNVGIDFNWEYPSSKHQHKKLVNRDLKTQSGSEMKKFLSTLTIDGVTRSDQGLYTCAASSGLQTKKNSTFVRVHEKDKTHTCPPCPAPEAAGGPSVFLFPPKPKDTLMISRTPEVTCVVVDVSHEDPEVKFNWYVDGVEVHNAKTKPREEQYNSTYRVVSVLTVLHQDWLNGKEYKCKVSNKALPAPIEKTISKAKGQPREPQVYTLPPSREEMTKNQVSLTCLVKGFYPSDIAVEWESNGQPENNYKTTPPVLDSDGSFFLYSKLTVDKSRWQQGNVFSCSVMHEALHNHYTQKSLSLSPGK

SEQ ID NO: 35 - protein, 642 aa, synthetic construct
  source 1..642: note = PR1131 (R1D2-R2D3-linker-R2D2(Y221N)-R2D3(M314Q)-Fc)
SDTGRPFVEMYSEIPEIIHMTEGRELVIPCRVTSPNITVTLKKFPLDTLIPDGKRIIWDSRKGFIISNATYKEIGLLTCEATVNGHLYKTNYLTHRQTNTIIDVVLSPSHGIELSVGEKLVLNCTARTELNVGIDFNWEYPSSKHQHKKLVNRDLKTQSGSEMKKFLSTLTIDGVTRSDQGLYTCAASSGLMTKKNSTFVRVHEKGGGGSSPFIASVSDQHGVVYITENKNKTVVIPCLGSISNLNVSLCARYPEKRFVPDGNRISWDSKKGFTIPSYMISYAGMVFCEAKINDESYQSIMYIVVVVGNRIYDVVLSPSHGIELSVGEKLVLNCTARTELNVGIDFNWEYPSSKHQHKKLVNRDLKTQSGSEMKKFLSTLTIDGVTRSDQGLYTCAASSGLQTKKNSTFVRVHEKDKTHTCPPCPAPEAAGGPSVFLFPPKPKDTLMISRTPEVTCVVVDVSHEDPEVKFNWYVDGVEVHNAKTKPREEQYNSTYRVVSVLTVLHQDWLNGKEYKCKVSNKALPAPIEKTISKAKGQPREPQVYTLPPSREEMTKNQVSLTCLVKGFYPSDIAVEWESNGQPENNYKTTPPVLDSDGSFFLYSKLTVDKSRWQQGNVFSCSVMHEALHNHYTQKSLSLSPGK

SEQ ID NO: 36 - protein, 642 aa, synthetic construct
  source 1..642: note = PR1132 (R1D2-R2D3-linker-R2D2-R2D3(L277R/L289Y)-Fc)
SDTGRPFVEMYSEIPEIIHMTEGRELVIPCRVTSPNITVTLKKFPLDTLIPDGKRIIWDSRKGFIISNATYKEIGLLTCEATVNGHLYKTNYLTHRQTNTIIDVVLSPSHGIELSVGEKLVLNCTARTELNVGIDFNWEYPSSKHQHKKLVNRDLKTQSGSEMKKFLSTLTIDGVTRSDQGLYTCAASSGLMTKKNSTFVRVHEKGGGGSSPFIASVSDQHGVVYITENKNKTVVIPCLGSISNLNVSLCARYPEKRFVPDGNRISWDSKKGFTIPSYMISYAGMVFCEAKINDESYQSIMYIVVVVGYRIYDVVLSPSHGIELSVGEKLVLNCTARTELNVGIDFNWEYPSSKHQHKKLVNRDRKTQSGSEMKKFYSTLTIDGVTRSDQGLYTCAASSGLMTKKNSTFVRVHEKDKTHTCPPCPAPEAAGGPSVFLFPPKPKDTLMISRTPEVTCVVVDVSHEDPEVKFNWYVDGVEVHNAKTKPREEQYNSTYRVVSVLTVLHQDWLNGKEYKCKVSNKALPAPIEKTISKAKGQPREPQVYTLPPSREEMTKNQVSLTCLVKGFYPSDIAVEWESNGQPENNYKTTPPVLDSDGSFFLYSKLTVDKSRWQQGNVFSCSVMHEALHNHYTQKSLSLSPGK

SEQ ID NO: 37 - protein, 642 aa, synthetic construct
  source 1..642: note = PR1135 (R1D2-R2D3-linker-R2D2(Y221S/R222K)-R2D3-Fc)
SDTGRPFVEMYSEIPEIIHMTEGRELVIPCRVTSPNITVTLKKFPLDTLIPDGKRIIWDSRKGFIISNATYKEIGLLTCEATVNGHLYKTNYLTHRQTNTIIDVVLSPSHGIELSVGEKLVLNCTARTELNVGIDFNWEYPSSKHQHKKLVNRDLKTQSGSEMKKFLSTLTIDGVTRSDQGLYTCAASSGLMTKKNSTFVRVHEKGGGGSSPFIASVSDQHGVVYITENKNKTVVIPCLGSISNLNVSLCARYPEKRFVPDGNRISWDSKKGFTIPSYMISYAGMVFCEAKINDESYQSIMYIVVVVGSKIYDVVLSPSHGIELSVGEKLVLNCTARTELNVGIDFNWEYPSSKHQHKKLVNRDLKTQSGSEMKKFLSTLTIDGVTRSDQGLYTCAASSGLMTKKNSTFVRVHEKDKTHTCPPCPAPEAAGGPSVFLFPPKPKDTLMISRTPEVTCVVVDVSHEDPEVKFNWYVDGVEVHNAKTKPREEQYNSTYRVVSVLTVLHQDWLNGKEYKCKVSNKALPAPIEKTISKAKGQPREPQVYTLPPSREEMTKNQVSLTCLVKGFYPSDIAVEWESNGQPENNYKTTPPVLDSDGSFFLYSKLTVDKSRWQQGNVFSCSVMHEALHNHYTQKSLSLSPGK

SEQ ID NO: 38 - protein, 642 aa, synthetic construct
  source 1..642: note = PR1136 (R1D2-R2D3-linker-R2D2-R2D3(L313R)-Fc)
SDTGRPFVEMYSEIPEIIHMTEGRELVIPCRVTSPNITVTLKKFPLDTLIPDGKRIIWDSRKGFIISNATYKEIGLLTCEATVNGHLYKTNYLTHRQTNTIIDVVLSPSHGIELSVGEKLVLNCTARTELNVGIDFNWEYPSSKHQHKKLVNRDLKTQSGSEMKKFLSTLTIDGVTRSDQGLYTCAASSGLMTKKNSTFVRVHEKGGGGSSPFIASVSDQHGVVYITENKNKTVVIPCLGSISNLNVSLCARYPEKRFVPDGNRISWDSKKGFTIPSYMISYAGMVFCEAKINDESYQSIMYIVVVVGYRIYDVVLSPSHGIELSVGEKLVLNCTARTELNVGIDFNWEYPSSKHQHKKLVNRDLKTQSGSEMKKFLSTLTIDGVTRSDQGLYTCAASSGRMTKKNSTFVRVHEKDKTHTCPPCPAPEAAGGPSVFLFPPKPKDTLMISRTPEVTCVVVDVSHEDPEVKFNWYVDGVEVHNAKTKPREEQYNSTYRVVSVLTVLHQDWLNGKEYKCKVSNKALPAPIEKTISKAKGQPREPQVYTLPPSREEMTKNQVSLTCLVKGFYPSDIAVEWESNGQPENNYKTTPPVLDSDGSFFLYSKLTVDKSRWQQGNVFSCSVMHEALHNHYTQKSLSLSPGK

SEQ ID NO: 39 - protein, 642 aa, synthetic construct
  source 1..642: note = PR1139 (R1D2-R2D3-linker-R2D2-R2D3(N245Q)-Fc)
SDTGRPFVEMYSEIPEIIHMTEGRELVIPCRVTSPNITVTLKKFPLDTLIPDGKRIIWDSRKGFIISNATYKEIGLLTCEATVNGHLYKTNYLTHRQTNTIIDVVLSPSHGIELSVGEKLVLNCTARTELNVGIDFNWEYPSSKHQHKKLVNRDLKTQSGSEMKKFLSTLTIDGVTRSDQGLYTCAASSGLMTKKNSTFVRVHEKGGGGSSPFIASVSDQHGVVYITENKNKTVVIPCLGSISNLNVSLCARYPEKRFVPDGNRISWDSKKGFTIPSYMISYAGMVFCEAKINDESYQSIMYIVVVVGYRIYDVVLSPSHGIELSVGEKLVLQCTARTELNVGIDFNWEYPSSKHQHKKLVNRDLKTQSGSEMKKFLSTLTIDGVTRSDQGLYTCAASSGLMTKKNSTFVRVHEKDKTHTCPPCPAPEAAGGPSVFLFPPKPKDTLMISRTPEVTCVVVDVSHEDPEVKFNWYVDGVEVHNAKTKPREEQYNSTYRVVSVLTVLHQDWLNGKEYKCKVSNKALPAPIEKTISKAKGQPREPQVYTLPPSREEMTKNQVSLTCLVKGFYPSDIAVEWESNGQPENNYKTTPPVLDSDGSFFLYSKLTVDKSRWQQGNVFSCSVMHEALHNHYTQKSLSLSPGK

SEQ ID NO: 40 - protein, 642 aa, synthetic construct
  source 1..642: note = PR1141 (R1D2-R2D3-linker-R2D2(C162V)-R2D3(N274F)-Fc)
SDTGRPFVEMYSEIPEIIHMTEGRELVIPCRVTSPNITVTLKKFPLDTLIPDGKRIIWDSRKGFIISNATYKEIGLLTCEATVNGHLYKTNYLTHRQTNTIIDVVLSPSHGIELSVGEKLVLNCTARTELNVGIDFNWEYPSSKHQHKKLVNRDLKTQSGSEMKKFLSTLTIDGVTRSDQGLYTCAASSGLMTKKNSTFVRVHEKGGGGSSPFIASVSDQHGVVYITENKNKTVVIPCLGSISNLNVSLVARYPEKRFVPDGNRISWDSKKGFTIPSYMISYAGMVFCEAKINDESYQSIMYIVVVVGYRIYDVVLSPSHGIELSVGEKLVLNCTARTELNVGIDFNWEYPSSKHQHKKLVFRDLKTQSGSEMKKFLSTLTIDGVTRSDQGLYTCAASSGLMTKKNSTFVRVHEKDKTHTCPPCPAPEAAGGPSVFLFPPKPKDTLMISRTPEVTCVVVDVSHEDPEVKFNWYVDGVEVHNAKTKPREEQYNSTYRVVSVLTVLHQDWLNGKEYKCKVSNKALPAPIEKTISKAKGQPREPQVYTLPPSREEMTKNQVSLTCLVKGFYPSDIAVEWESNGQPENNYKTTPPVLDSDGSFFLYSKLTVDKSRWQQGNVFSCSVMHEALHNHYTQKSLSLSPGK

SEQ ID NO: 41 - protein, 642 aa, synthetic construct
  source 1..642: note = PR1142 (R1D2-R2D3-linker-R2D2(C162V)-R2D3(N274I)-Fc)
SDTGRPFVEMYSEIPEIIHMTEGRELVIPCRVTSPNITVTLKKFPLDTLIPDGKRIIWDSRKGFIISNATYKEIGLLTCEATVNGHLYKTNYLTHRQTNTIIDVVLSPSHGIELSVGEKLVLNCTARTELNVGIDFNWEYPSSKHQHKKLVNRDLKTQSGSEMKKFLSTLTIDGVTRSDQGLYTCAASSGLMTKKNSTFVRVHEKGGGGSSPFIASVSDQHGVVYITENKNKTVVIPCLGSISNLNVSLVARYPEKRFVPDGNRISWDSKKGFTIPSYMISYAGMVFCEAKINDESYQSIMYIVVVVGYRIYDVVLSPSHGIELSVGEKLVLNCTARTELNVGIDFNWEYPSSKHQHKKLVIRDLKTQSGSEMKKFLSTLTIDGVTRSDQGLYTCAASSGLMTKKNSTFVRVHEKDKTHTCPPCPAPEAAGGPSVFLFPPKPKDTLMISRTPEVTCVVVDVSHEDPEVKFNWYVDGVEVHNAKTKPREEQYNSTYRVVSVLTVLHQDWLNGKEYKCKVSNKALPAPIEKTISKAKGQPREPQVYTLPPSREEMTKNQVSLTCLVKGFYPSDIAVEWESNGQPENNYKTTPPVLDSDGSFFLYSKLTVDKSRWQQGNVFSCSVMHEALHNHYTQKSLSLSPGK

SEQ ID NO: 42 - protein, 642 aa, synthetic construct
  source 1..642: note = PR1143 (R1D2-R2D3-linker-R2D2(C162V)-R2D3(R275L)-Fc)
SDTGRPFVEMYSEIPEIIHMTEGRELVIPCRVTSPNITVTLKKFPLDTLIPDGKRIIWDSRKGFIISNATYKEIGLLTCEATVNGHLYKTNYLTHRQTNTIIDVVLSPSHGIELSVGEKLVLNCTARTELNVGIDFNWEYPSSKHQHKKLVNRDLKTQSGSEMKKFLSTLTIDGVTRSDQGLYTCAASSGLMTKKNSTFVRVHEKGGGGSSPFIASVSDQHGVVYITENKNKTVVIPCLGSISNLNVSLVARYPEKRFVPDGNRISWDSKKGFTIPSYMISYAGMVFCEAKINDESYQSIMYIVVVVGYRIYDVVLSPSHGIELSVGEKLVLNCTARTELNVGIDFNWEYPSSKHQHKKLVNLDLKTQSGSEMKKFLSTLTIDGVTRSDQGLYTCAASSGLMTKKNSTFVRVHEKDKTHTCPPCPAPEAAGGPSVFLFPPKPKDTLMISRTPEVTCVVVDVSHEDPEVKFNWYVDGVEVHNAKTKPREEQYNSTYRVVSVLTVLHQDWLNGKEYKCKVSNKALPAPIEKTISKAKGQPREPQVYTLPPSREEMTKNQVSLTCLVKGFYPSDIAVEWESNGQPENNYKTTPPVLDSDGSFFLYSKLTVDKSRWQQGNVFSCSVMHEALHNHYTQKSLSLSPGK

SEQ ID NO: 43 - protein, 642 aa, synthetic construct
  source 1..642: note = PR1144 (R1D2-R2D3-linker-R2D2(C162V)-R2D3(D276Q)-Fc)
SDTGRPFVEMYSEIPEIIHMTEGRELVIPCRVTSPNITVTLKKFPLDTLIPDGKRIIWDSRKGFIISNATYKEIGLLTCEATVNGHLYKTNYLTHRQTNTIIDVVLSPSHGIELSVGEKLVLNCTARTELNVGIDFNWEYPSSKHQHKKLVNRDLKTQSGSEMKKFLSTLTIDGVTRSDQGLYTCAASSGLMTKKNSTFVRVHEKGGGGSSPFIASVSDQHGVVYITENKNKTVVIPCLGSISNLNVSLVARYPEKRFVPDGNRISWDSKKGFTIPSYMISYAGMVFCEAKINDESYQSIMYIVVVVGYRIYDVVLSPSHGIELSVGEKLVLNCTARTELNVGIDFNWEYPSSKHQHKKLVNRQLKTQSGSEMKKFLSTLTIDGVTRSDQGLYTCAASSGLMTKKNSTFVRVHEKDKTHTCPPCPAPEAAGGPSVFLFPPKPKDTLMISRTPEVTCVVVDVSHEDPEVKFNWYVDGVEVHNAKTKPREEQYNSTYRVVSVLTVLHQDWLNGKEYKCKVSNKALPAPIEKTISKAKGQPREPQVYTLPPSREEMTKNQVSLTCLVKGFYPSDIAVEWESNGQPENNYKTTPPVLDSDGSFFLYSKLTVDKSRWQQGNVFSCSVMHEALHNHYTQKSLSLSPGK

SEQ ID NO: 44 - protein, 642 aa, synthetic construct
  source 1..642: note = PR1145 (R1D2-R2D3-linker-R2D2(C162V)-R2D3(S283T)-Fc)
SDTGRPFVEMYSEIPEIIHMTEGRELVIPCRVTSPNITVTLKKFPLDTLIPDGKRIIWDSRKGFIISNATYKEIGLLTCEATVNGHLYKTNYLTHRQTNTIIDVVLSPSHGIELSVGEKLVLNCTARTELNVGIDFNWEYPSSKHQHKKLVNRDLKTQSGSEMKKFLSTLTIDGVTRSDQGLYTCAASSGLMTKKNSTFVRVHEKGGGGSSPFIASVSDQHGVVYITENKNKTVVIPCLGSISNLNVSLVARYPEKRFVPDGNRISWDSKKGFTIPSYMISYAGMVFCEAKINDESYQSIMYIVVVVGYRIYDVVLSPSHGIELSVGEKLVLNCTARTELNVGIDFNWEYPSSKHQHKKLVNRDLKTQSGTEMKKFLSTLTIDGVTRSDQGLYTCAASSGLMTKKNSTFVRVHEKDKTHTCPPCPAPEAAGGPSVFLFPPKPKDTLMISRTPEVTCVVVDVSHEDPEVKFNWYVDGVEVHNAKTKPREEQYNSTYRVVSVLTVLHQDWLNGKEYKCKVSNKALPAPIEKTISKAKGQPREPQVYTLPPSREEMTKNQVSLTCLVKGFYPSDIAVEWESNGQPENNYKTTPPVLDSDGSFFLYSKLTVDKSRWQQGNVFSCSVMHEALHNHYTQKSLSLSPGK

SEQ ID NO: 45 - protein, 642 aa, synthetic construct
  source 1..642: note = PR1146 (R1D2-R2D3-linker-R2D2(C162V)-R2D3(L289Y)-Fc)
SDTGRPFVEMYSEIPEIIHMTEGRELVIPCRVTSPNITVTLKKFPLDTLIPDGKRIIWDSRKGFIISNATYKEIGLLTCEATVNGHLYKTNYLTHRQTNTIIDVVLSPSHGIELSVGEKLVLNCTARTELNVGIDFNWEYPSSKHQHKKLVNRDLKTQSGSEMKKFLSTLTIDGVTRSDQGLYTCAASSGLMTKKNSTFVRVHEKGGGGSSPFIASVSDQHGVVYITENKNKTVVIPCLGSISNLNVSLVARYPEKRFVPDGNRISWDSKKGFTIPSYMISYAGMVFCEAKINDESYQSIMYIVVVVGYRIYDVVLSPSHGIELSVGEKLVLNCTARTELNVGIDFNWEYPSSKHQHKKLVNRDLKTQSGSEMKKFYSTLTIDGVTRSDQGLYTCAASSGLMTKKNSTFVRVHEKDKTHTCPPCPAPEAAGGPSVFLFPPKPKDTLMISRTPEVTCVVVDVSHEDPEVKFNWYVDGVEVHNAKTKPREEQYNSTYRVVSVLTVLHQDWLNGKEYKCKVSNKALPAPIEKTISKAKGQPREPQVYTLPPSREEMTKNQVSLTCLVKGFYPSDIAVEWESNGQPENNYKTTPPVLDSDGSFFLYSKLTVDKSRWQQGNVFSCSVMHEALHNHYTQKSLSLSPGK

SEQ ID NO: 46 - protein, 642 aa, synthetic construct
  source 1..642: note = PR1147 (R1D2-R2D3-linker-R2D2(C162V)-R2D3(L313Y)-Fc)
SDTGRPFVEMYSEIPEIIHMTEGRELVIPCRVTSPNITVTLKKFPLDTLIPDGKRIIWDSRKGFIISNATYKEIGLLTCEATVNGHLYKTNYLTHRQTNTIIDVVLSPSHGIELSVGEKLVLNCTARTELNVGIDFNWEYPSSKHQHKKLVNRDLKTQSGSEMKKFLSTLTIDGVTRSDQGLYTCAASSGLMTKKNSTFVRVHEKGGGGSSPFIASVSDQHGVVYITENKNKTVVIPCLGSISNLNVSLVARYPEKRFVPDGNRISWDSKKGFTIPSYMISYAGMVFCEAKINDESYQSIMYIVVVVGYRIYDVVLSPSHGIELSVGEKLVLNCTARTELNVGIDFNWEYPSSKHQHKKLVNRDLKTQSGSEMKKFLSTLTIDGVTRSDQGLYTCAASSGYMTKKNSTFVRVHEKDKTHTCPPCPAPEAAGGPSVFLFPPKPKDTLMISRTPEVTCVVVDVSHEDPEVKFNWYVDGVEVHNAKTKPREEQYNSTYRVVSVLTVLHQDWLNGKEYKCKVSNKALPAPIEKTISKAKGQPREPQVYTLPPSREEMTKNQVSLTCLVKGFYPSDIAVEWESNGQPENNYKTTPPVLDSDGSFFLYSKLTVDKSRWQQGNVFSCSVMHEALHNHYTQKSLSLSPGK

SEQ ID NO: 47 - protein, 642 aa, synthetic construct
  source 1..642: note = PR1148 (R1D2-R2D3-linker-R2D2(C162V)-R2D3(L277R/L289Y)-Fc)
SDTGRPFVEMYSEIPEIIHMTEGRELVIPCRVTSPNITVTLKKFPLDTLIPDGKRIIWDSRKGFIISNATYKEIGLLTCEATVNGHLYKTNYLTHRQTNTIIDVVLSPSHGIELSVGEKLVLNCTARTELNVGIDFNWEYPSSKHQHKKLVNRDLKTQSGSEMKKFLSTLTIDGVTRSDQGLYTCAASSGLMTKKNSTFVRVHEKGGGGSSPFIASVSDQHGVVYITENKNKTVVIPCLGSISNLNVSLVARYPEKRFVPDGNRISWDSKKGFTIPSYMISYAGMVFCEAKINDESYQSIMYIVVVVGYRIYDVVLSPSHGIELSVGEKLVLNCTARTELNVGIDFNWEYPSSKHQHKKLVNRDRKTQSGSEMKKFYSTLTIDGVTRSDQGLYTCAASSGLMTKKNSTFVRVHEKDKTHTCPPCPAPEAAGGPSVFLFPPKPKDTLMISRTPEVTCVVVDVSHEDPEVKFNWYVDGVEVHNAKTKPREEQYNSTYRVVSVLTVLHQDWLNGKEYKCKVSNKALPAPIEKTISKAKGQPREPQVYTLPPSREEMTKNQVSLTCLVKGFYPSDIAVEWESNGQPENNYKTTPPVLDSDGSFFLYSKLTVDKSRWQQGNVFSCSVMHEALHNHYTQKSLSLSPGK

SEQ ID NO: 48 - protein, 642 aa, synthetic construct
  source 1..642: note = PR1149 (R1D2-R2D3-linker-R2D2(C162V/Y221S/R222K)-R2D3-Fc)
SDTGRPFVEMYSEIPEIIHMTEGRELVIPCRVTSPNITVTLKKFPLDTLIPDGKRIIWDSRKGFIISNATYKEIGLLTCEATVNGHLYKTNYLTHRQTNTIIDVVLSPSHGIELSVGEKLVLNCTARTELNVGIDFNWEYPSSKHQHKKLVNRDLKTQSGSEMKKFLSTLTIDGVTRSDQGLYTCAASSGLMTKKNSTFVRVHEKGGGGSSPFIASVSDQHGVVYITENKNKTVVIPCLGSISNLNVSLVARYPEKRFVPDGNRISWDSKKGFTIPSYMISYAGMVFCEAKINDESYQSIMYIVVVVGSKIYDVVLSPSHGIELSVGEKLVLNCTARTELNVGIDFNWEYPSSKHQHKKLVNRDLKTQSGSEMKKFLSTLTIDGVTRSDQGLYTCAASSGLMTKKNSTFVRVHEKDKTHTCPPCPAPEAAGGPSVFLFPPKPKDTLMISRTPEVTCVVVDVSHEDPEVKFNWYVDGVEVHNAKTKPREEQYNSTYRVVSVLTVLHQDWLNGKEYKCKVSNKALPAPIEKTISKAKGQPREPQVYTLPPSREEMTKNQVSLTCLVKGFYPSDIAVEWESNGQPENNYKTTPPVLDSDGSFFLYSKLTVDKSRWQQGNVFSCSVMHEALHNHYTQKSLSLSPGK

SEQ ID NO: 49 - protein, 642 aa, synthetic construct
  source 1..642: note = PR1150 (R1D2-R2D3-linker-R2D2(C162V)-R2D3(L313R)-Fc)
SDTGRPFVEMYSEIPEIIHMTEGRELVIPCRVTSPNITVTLKKFPLDTLIPDGKRIIWDSRKGFIISNATYKEIGLLTCEATVNGHLYKTNYLTHRQTNTIIDVVLSPSHGIELSVGEKLVLNCTARTELNVGIDFNWEYPSSKHQHKKLVNRDLKTQSGSEMKKFLSTLTIDGVTRSDQGLYTCAASSGLMTKKNSTFVRVHEKGGGGSSPFIASVSDQHGVVYITENKNKTVVIPCLGSISNLNVSLVARYPEKRFVPDGNRISWDSKKGFTIPSYMISYAGMVFCEAKINDESYQSIMYIVVVVGYRIYDVVLSPSHGIELSVGEKLVLNCTARTELNVGIDFNWEYPSSKHQHKKLVNRDLKTQSGSEMKKFLSTLTIDGVTRSDQGLYTCAASSGRMTKKNSTFVRVHEKDKTHTCPPCPAPEAAGGPSVFLFPPKPKDTLMISRTPEVTCVVVDVSHEDPEVKFNWYVDGVEVHNAKTKPREEQYNSTYRVVSVLTVLHQDWLNGKEYKCKVSNKALPAPIEKTISKAKGQPREPQVYTLPPSREEMTKNQVSLTCLVKGFYPSDIAVEWESNGQPENNYKTTPPVLDSDGSFFLYSKLTVDKSRWQQGNVFSCSVMHEALHNHYTQKSLSLSPGK

SEQ ID NO: 50 - protein, 677 aa, synthetic construct
  source 1..677: note = PR1163 (heavy chain: R2D2(C162V)-R2D3-Fc-linker-VH-CH1)
SPFIASVSDQHGVVYITENKNKTVVIPCLGSISNLNVSLVARYPEKRFVPDGNRISWDSKKGFTIPSYMISYAGMVFCEAKINDESYQSIMYIVVVVGYRIYDVVLSPSHGIELSVGEKLVLNCTARTELNVGIDFNWEYPSSKHQHKKLVNRDLKTQSGSEMKKFLSTLTIDGVTRSDQGLYTCAASSGLMTKKNSTFVRVHEKDKTHTCPPCPAPEAAGGPSVFLFPPKPKDTLMISRTPEVTCVVVDVSHEDPEVKFNWYVDGVEVHNAKTKPREEQYNSTYRVVSVLTVLHQDWLNGKEYKCKVSNKALPAPIEKTISKAKGQPREPQVYTLPPSREEMTKNQVSLTCLVKGFYPSDIAVEWESNGQPENNYKTTPPVLDSDGSFFLYSKLTVDKSRWQQGNVFSCSVMHEALHNHYTQKSLSLSPGGGGGSGGGGSGGGGSGGGGSEVQLVESGGGLVQPGGSLRLSCAASGYTFTNYGMNWVRQAPGKGLEWVGWINTYTGEPTYAADFKRRFTFSLDTSKSTAYLQMNSLRAEDTAVYYCAKYPHYYGSSHWYFDVWGQGTLVTVSSASTKGPSVFPLAPSSKSTSGGTAALGCLVKDYFPEPVTVSWNSGALTSGVHTFPAVLQSSGLYSLSSVVTVPSSSLGTQTYICNVNHKPSNTKVDKKVEPKSC

SEQ ID NO: 51 - protein, 214 aa, synthetic construct
  source 1..214: note = PR1163 light chain L: VL-CL
DIQMTQSPSSLSASVGDRVTITCSASQDISNYLNWYQQKPGKAPKVLIYFTSSLHSGVPSRFSGSGSGTDFTLTISSLQPEDFATYYCQQYSTVPWTFGQGTKVEIKRTVAAPSVFIFPPSDEQLKSGTASVVCLLNNFYPREAKVQWKVDNALQSGNSQESVTEQDSKDSTYSLSSTLTLSKADYEKHKVYACEVTHQGLSSPVTKSFNRGEC

SEQ ID NO: 52 - protein, 642 aa, synthetic construct
  source 1..642: note = PR1165 (R1D2-R2D3-linker-R2D2(C162I)-R2D3-Fc)
SDTGRPFVEMYSEIPEIIHMTEGRELVIPCRVTSPNITVTLKKFPLDTLIPDGKRIIWDSRKGFIISNATYKEIGLLTCEATVNGHLYKTNYLTHRQTNTIIDVVLSPSHGIELSVGEKLVLNCTARTELNVGIDFNWEYPSSKHQHKKLVNRDLKTQSGSEMKKFLSTLTIDGVTRSDQGLYTCAASSGLMTKKNSTFVRVHEKGGGGSSPFIASVSDQHGVVYITENKNKTVVIPCLGSISNLNVSLIARYPEKRFVPDGNRISWDSKKGFTIPSYMISYAGMVFCEAKINDESYQSIMYIVVVVGYRIYDVVLSPSHGIELSVGEKLVLNCTARTELNVGIDFNWEYPSSKHQHKKLVNRDLKTQSGSEMKKFLSTLTIDGVTRSDQGLYTCAASSGLMTKKNSTFVRVHEKDKTHTCPPCPAPEAAGGPSVFLFPPKPKDTLMISRTPEVTCVVVDVSHEDPEVKFNWYVDGVEVHNAKTKPREEQYNSTYRVVSVLTVLHQDWLNGKEYKCKVSNKALPAPIEKTISKAKGQPREPQVYTLPPSREEMTKNQVSLTCLVKGFYPSDIAVEWESNGQPENNYKTTPPVLDSDGSFFLYSKLTVDKSRWQQGNVFSCSVMHEALHNHYTQKSLSLSPGK

SEQ ID NO: 53 - protein, 642 aa, synthetic construct
  source 1..642: note = PR1166 (R1D2-R2D3-linker-R2D2(C162L)-R2D3-Fc)
SDTGRPFVEMYSEIPEIIHMTEGRELVIPCRVTSPNITVTLKKFPLDTLIPDGKRIIWDSRKGFIISNATYKEIGLLTCEATVNGHLYKTNYLTHRQTNTIIDVVLSPSHGIELSVGEKLVLNCTARTELNVGIDFNWEYPSSKHQHKKLVNRDLKTQSGSEMKKFLSTLTIDGVTRSDQGLYTCAASSGLMTKKNSTFVRVHEKGGGGSSPFIASVSDQHGVVYITENKNKTVVIPCLGSISNLNVSLLARYPEKRFVPDGNRISWDSKKGFTIPSYMISYAGMVFCEAKINDESYQSIMYIVVVVGYRIYDVVLSPSHGIELSVGEKLVLNCTARTELNVGIDFNWEYPSSKHQHKKLVNRDLKTQSGSEMKKFLSTLTIDGVTRSDQGLYTCAASSGLMTKKNSTFVRVHEKDKTHTCPPCPAPEAAGGPSVFLFPPKPKDTLMISRTPEVTCVVVDVSHEDPEVKFNWYVDGVEVHNAKTKPREEQYNSTYRVVSVLTVLHQDWLNGKEYKCKVSNKALPAPIEKTISKAKGQPREPQVYTLPPSREEMTKNQVSLTCLVKGFYPSDIAVEWESNGQPENNYKTTPPVLDSDGSFFLYSKLTVDKSRWQQGNVFSCSVMHEALHNHYTQKSLSLSPGK

SEQ ID NO: 54 - protein, 637 aa, synthetic construct
  source 1..637: note = PR1167 (R1D2-R2D3-R2D2(C162V)-R2D3(N274F/S283T)-Fc)
SDTGRPFVEMYSEIPEIIHMTEGRELVIPCRVTSPNITVTLKKFPLDTLIPDGKRIIWDSRKGFIISNATYKEIGLLTCEATVNGHLYKTNYLTHRQTNTIIDVVLSPSHGIELSVGEKLVLNCTARTELNVGIDFNWEYPSSKHQHKKLVNRDLKTQSGSEMKKFLSTLTIDGVTRSDQGLYTCAASSGLMTKKNSTFVRVHEKSPFIASVSDQHGVVYITENKNKTVVIPCLGSISNLNVSLVARYPEKRFVPDGNRISWDSKKGFTIPSYMISYAGMVFCEAKINDESYQSIMYIVVVVGYRIYDVVLSPSHGIELSVGEKLVLNCTARTELNVGIDFNWEYPSSKHQHKKLVFRDLKTQSGTEMKKFLSTLTIDGVTRSDQGLYTCAASSGLMTKKNSTFVRVHEKDKTHTCPPCPAPEAAGGPSVFLFPPKPKDTLMISRTPEVTCVVVDVSHEDPEVKFNWYVDGVEVHNAKTKPREEQYNSTYRVVSVLTVLHQDWLNGKEYKCKVSNKALPAPIEKTISKAKGQPREPQVYTLPPSREEMTKNQVSLTCLVKGFYPSDIAVEWESNGQPENNYKTTPPVLDSDGSFFLYSKLTVDKSRWQQGNVFSCSVMHEALHNHYTQKSLSLSPGK

SEQ ID NO: 55 - protein, 637 aa, synthetic construct
  source 1..637: note = PR1168 (R1D2-R2D3-R2D2(C162V/Y221S/R222K)-R2D3(N274F)-Fc)
SDTGRPFVEMYSEIPEIIHMTEGRELVIPCRVTSPNITVTLKKFPLDTLIPDGKRIIWDSRKGFIISNATYKEIGLLTCEATVNGHLYKTNYLTHRQTNTIIDVVLSPSHGIELSVGEKLVLNCTARTELNVGIDFNWEYPSSKHQHKKLVNRDLKTQSGSEMKKFLSTLTIDGVTRSDQGLYTCAASSGLMTKKNSTFVRVHEKSPFIASVSDQHGVVYITENKNKTVVIPCLGSISNLNVSLVARYPEKRFVPDGNRISWDSKKGFTIPSYMISYAGMVFCEAKINDESYQSIMYIVVVVGSKIYDVVLSPSHGIELSVGEKLVLNCTARTELNVGIDFNWEYPSSKHQHKKLVFRDLKTQSGSEMKKFLSTLTIDGVTRSDQGLYTCAASSGLMTKKNSTFVRVHEKDKTHTCPPCPAPEAAGGPSVFLFPPKPKDTLMISRTPEVTCVVVDVSHEDPEVKFNWYVDGVEVHNAKTKPREEQYNSTYRVVSVLTVLHQDWLNGKEYKCKVSNKALPAPIEKTISKAKGQPREPQVYTLPPSREEMTKNQVSLTCLVKGFYPSDIAVEWESNGQPENNYKTTPPVLDSDGSFFLYSKLTVDKSRWQQGNVFSCSVMHEALHNHYTQKSLSLSPGK

SEQ ID NO: 56 - protein, 637 aa, synthetic construct
  source 1..637: note = PR1169 (R1D2-R2D3-R2D2(C162V/Y221S/R222K)-R2D3(S283T)-Fc)
SDTGRPFVEMYSEIPEIIHMTEGRELVIPCRVTSPNITVTLKKFPLDTLIPDGKRIIWDSRKGFIISNATYKEIGLLTCEATVNGHLYKTNYLTHRQTNTIIDVVLSPSHGIELSVGEKLVLNCTARTELNVGIDFNWEYPSSKHQHKKLVNRDLKTQSGSEMKKFLSTLTIDGVTRSDQGLYTCAASSGLMTKKNSTFVRVHEKSPFIASVSDQHGVVYITENKNKTVVIPCLGSISNLNVSLVARYPEKRFVPDGNRISWDSKKGFTIPSYMISYAGMVFCEAKINDESYQSIMYIVVVVGSKIYDVVLSPSHGIELSVGEKLVLNCTARTELNVGIDFNWEYPSSKHQHKKLVNRDLKTQSGTEMKKFLSTLTIDGVTRSDQGLYTCAASSGLMTKKNSTFVRVHEKDKTHTCPPCPAPEAAGGPSVFLFPPKPKDTLMISRTPEVTCVVVDVSHEDPEVKFNWYVDGVEVHNAKTKPREEQYNSTYRVVSVLTVLHQDWLNGKEYKCKVSNKALPAPIEKTISKAKGQPREPQVYTLPPSREEMTKNQVSLTCLVKGFYPSDIAVEWESNGQPENNYKTTPPVLDSDGSFFLYSKLTVDKSRWQQGNVFSCSVMHEALHNHYTQKSLSLSPGK

SEQ ID NO: 57 - protein, 637 aa, synthetic construct
  source 1..637: note = PR1170 (R1D2-R2D3-R2D2(C162V/Y221S/R222K)-R2D3(N274F/S283T)-Fc)
SDTGRPFVEMYSEIPEIIHMTEGRELVIPCRVTSPNITVTLKKFPLDTLIPDGKRIIWDSRKGFIISNATYKEIGLLTCEATVNGHLYKTNYLTHRQTNTIIDVVLSPSHGIELSVGEKLVLNCTARTELNVGIDFNWEYPSSKHQHKKLVNRDLKTQSGSEMKKFLSTLTIDGVTRSDQGLYTCAASSGLMTKKNSTFVRVHEKSPFIASVSDQHGVVYITENKNKTVVIPCLGSISNLNVSLVARYPEKRFVPDGNRISWDSKKGFTIPSYMISYAGMVFCEAKINDESYQSIMYIVVVVGSKIYDVVLSPSHGIELSVGEKLVLNCTARTELNVGIDFNWEYPSSKHQHKKLVFRDLKTQSGTEMKKFLSTLTIDGVTRSDQGLYTCAASSGLMTKKNSTFVRVHEKDKTHTCPPCPAPEAAGGPSVFLFPPKPKDTLMISRTPEVTCVVVDVSHEDPEVKFNWYVDGVEVHNAKTKPREEQYNSTYRVVSVLTVLHQDWLNGKEYKCKVSNKALPAPIEKTISKAKGQPREPQVYTLPPSREEMTKNQVSLTCLVKGFYPSDIAVEWESNGQPENNYKTTPPVLDSDGSFFLYSKLTVDKSRWQQGNVFSCSVMHEALHNHYTQKSLSLSPGK

SEQ ID NO: 58 - protein, 642 aa, synthetic construct
  source 1..642: note = PR1171 (R1D2-R2D3-linker-R2D2(C162V)-R2D3(N274F/S283T)-Fc)
SDTGRPFVEMYSEIPEIIHMTEGRELVIPCRVTSPNITVTLKKFPLDTLIPDGKRIIWDSRKGFIISNATYKEIGLLTCEATVNGHLYKTNYLTHRQTNTIIDVVLSPSHGIELSVGEKLVLNCTARTELNVGIDFNWEYPSSKHQHKKLVNRDLKTQSGSEMKKFLSTLTIDGVTRSDQGLYTCAASSGLMTKKNSTFVRVHEKGGGGSSPFIASVSDQHGVVYITENKNKTVVIPCLGSISNLNVSLVARYPEKRFVPDGNRISWDSKKGFTIPSYMISYAGMVFCEAKINDESYQSIMYIVVVVGYRIYDVVLSPSHGIELSVGEKLVLNCTARTELNVGIDFNWEYPSSKHQHKKLVFRDLKTQSGTEMKKFLSTLTIDGVTRSDQGLYTCAASSGLMTKKNSTFVRVHEKDKTHTCPPCPAPEAAGGPSVFLFPPKPKDTLMISRTPEVTCVVVDVSHEDPEVKFNWYVDGVEVHNAKTKPREEQYNSTYRVVSVLTVLHQDWLNGKEYKCKVSNKALPAPIEKTISKAKGQPREPQVYTLPPSREEMTKNQVSLTCLVKGFYPSDIAVEWESNGQPENNYKTTPPVLDSDGSFFLYSKLTVDKSRWQQGNVFSCSVMHEALHNHYTQKSLSLSPGK

SEQ ID NO: 59 - protein, 642 aa, synthetic construct
  source 1..642: note = PR1172 (R1D2-R2D3-linker-R2D2(C162V/Y221S/R222K)-R2D3(N274F)-Fc)
SDTGRPFVEMYSEIPEIIHMTEGRELVIPCRVTSPNITVTLKKFPLDTLIPDGKRIIWDSRKGFIISNATYKEIGLLTCEATVNGHLYKTNYLTHRQTNTIIDVVLSPSHGIELSVGEKLVLNCTARTELNVGIDFNWEYPSSKHQHKKLVNRDLKTQSGSEMKKFLSTLTIDGVTRSDQGLYTCAASSGLMTKKNSTFVRVHEKGGGGSSPFIASVSDQHGVVYITENKNKTVVIPCLGSISNLNVSLVARYPEKRFVPDGNRISWDSKKGFTIPSYMISYAGMVFCEAKINDESYQSIMYIVVVVGSKIYDVVLSPSHGIELSVGEKLVLNCTARTELNVGIDFNWEYPSSKHQHKKLVFRDLKTQSGSEMKKFLSTLTIDGVTRSDQGLYTCAASSGLMTKKNSTFVRVHEKDKTHTCPPCPAPEAAGGPSVFLFPPKPKDTLMISRTPEVTCVVVDVSHEDPEVKFNWYVDGVEVHNAKTKPREEQYNSTYRVVSVLTVLHQDWLNGKEYKCKVSNKALPAPIEKTISKAKGQPREPQVYTLPPSREEMTKNQVSLTCLVKGFYPSDIAVEWESNGQPENNYKTTPPVLDSDGSFFLYSKLTVDKSRWQQGNVFSCSVMHEALHNHYTQKSLSLSPGK

SEQ ID NO: 60 - protein, 642 aa, synthetic construct
  source 1..642: note = PR1173 (R1D2-R2D3-linker-R2D2(C162V/Y221S/R222K)-R2D3(S283T)-Fc)
SDTGRPFVEMYSEIPEIIHMTEGRELVIPCRVTSPNITVTLKKFPLDTLIPDGKRIIWDSRKGFIISNATYKEIGLLTCEATVNGHLYKTNYLTHRQTNTIIDVVLSPSHGIELSVGEKLVLNCTARTELNVGIDFNWEYPSSKHQHKKLVNRDLKTQSGSEMKKFLSTLTIDGVTRSDQGLYTCAASSGLMTKKNSTFVRVHEKGGGGSSPFIASVSDQHGVVYITENKNKTVVIPCLGSISNLNVSLVARYPEKRFVPDGNRISWDSKKGFTIPSYMISYAGMVFCEAKINDESYQSIMYIVVVVGSKIYDVVLSPSHGIELSVGEKLVLNCTARTELNVGIDFNWEYPSSKHQHKKLVNRDLKTQSGTEMKKFLSTLTIDGVTRSDQGLYTCAASSGLMTKKNSTFVRVHEKDKTHTCPPCPAPEAAGGPSVFLFPPKPKDTLMISRTPEVTCVVVDVSHEDPEVKFNWYVDGVEVHNAKTKPREEQYNSTYRVVSVLTVLHQDWLNGKEYKCKVSNKALPAPIEKTISKAKGQPREPQVYTLPPSREEMTKNQVSLTCLVKGFYPSDIAVEWESNGQPENNYKTTPPVLDSDGSFFLYSKLTVDKSRWQQGNVFSCSVMHEALHNHYTQKSLSLSPGK

SEQ ID NO: 61 - protein, 642 aa, synthetic construct
  source 1..642: note = PR1174 R1D2-R2D3-linker-R2D2(C162V/Y221S/R222K)- R2D3(N274F/S283T)-Fc
SDTGRPFVEMYSEIPEIIHMTEGRELVIPCRVTSPNITVTLKKFPLDTLIPDGKRIIWDSRKGFIISNATYKEIGLLTCEATVNGHLYKTNYLTHRQTNTIIDVVLSPSHGIELSVGEKLVLNCTARTELNVGIDFNWEYPSSKHQHKKLVNRDLKTQSGSEMKKFLSTLTIDGVTRSDQGLYTCAASSGLMTKKNSTFVRVHEKGGGGSSPFIASVSDQHGVVYITENKNKTVVIPCLGSISNLNVSLVARYPEKRFVPDGNRISWDSKKGFTIPSYMISYAGMVFCEAKINDESYQSIMYIVVVVGSKIYDVVLSPSHGIELSVGEKLVLNCTARTELNVGIDFNWEYPSSKHQHKKLVFRDLKTQSGTEMKKFLSTLTIDGVTRSDQGLYTCAASSGLMTKKNSTFVRVHEKDKTHTCPPCPAPEAAGGPSVFLFPPKPKDTLMISRTPEVTCVVVDVSHEDPEVKFNWYVDGVEVHNAKTKPREEQYNSTYRVVSVLTVLHQDWLNGKEYKCKVSNKALPAPIEKTISKAKGQPREPQVYTLPPSREEMTKNQVSLTCLVKGFYPSDIAVEWESNGQPENNYKTTPPVLDSDGSFFLYSKLTVDKSRWQQGNVFSCSVMHEALHNHYTQKSLSLSPGK

SEQ ID NO: 62 - protein, 432 aa, synthetic construct
  source 1..432: note = PR1175 (R2D2(C162V)-R2D3(N274F/S283T)-Fc)
SPFIASVSDQHGVVYITENKNKTVVIPCLGSISNLNVSLVARYPEKRFVPDGNRISWDSKKGFTIPSYMISYAGMVFCEAKINDESYQSIMYIVVVVGYRIYDVVLSPSHGIELSVGEKLVLNCTARTELNVGIDFNWEYPSSKHQHKKLVFRDLKTQSGTEMKKFLSTLTIDGVTRSDQGLYTCAASSGLMTKKNSTFVRVHEKDKTHTCPPCPAPEAAGGPSVFLFPPKPKDTLMISRTPEVTCVVVDVSHEDPEVKFNWYVDGVEVHNAKTKPREEQYNSTYRVVSVLTVLHQDWLNGKEYKCKVSNKALPAPIEKTISKAKGQPREPQVYTLPPSREEMTKNQVSLTCLVKGFYPSDIAVEWESNGQPENNYKTTPPVLDSDGSFFLYSKLTVDKSRWQQGNVFSCSVMHEALHNHYTQKSLSLSPGK

SEQ ID NO: 63 - protein, 432 aa, synthetic construct
  source 1..432: note = PR1176 (R2D2(C162V/Y221S/R222K)-R2D3(N274F)-Fc)
SPFIASVSDQHGVVYITENKNKTVVIPCLGSISNLNVSLVARYPEKRFVPDGNRISWDSKKGFTIPSYMISYAGMVFCEAKINDESYQSIMYIVVVVGSKIYDVVLSPSHGIELSVGEKLVLNCTARTELNVGIDFNWEYPSSKHQHKKLVFRDLKTQSGSEMKKFLSTLTIDGVTRSDQGLYTCAASSGLMTKKNSTFVRVHEKDKTHTCPPCPAPEAAGGPSVFLFPPKPKDTLMISRTPEVTCVVVDVSHEDPEVKFNWYVDGVEVHNAKTKPREEQYNSTYRVVSVLTVLHQDWLNGKEYKCKVSNKALPAPIEKTISKAKGQPREPQVYTLPPSREEMTKNQVSLTCLVKGFYPSDIAVEWESNGQPENNYKTTPPVLDSDGSFFLYSKLTVDKSRWQQGNVFSCSVMHEALHNHYTQKSLSLSPGK

SEQ ID NO: 64 - protein, 432 aa, synthetic construct
  source 1..432: note = PR1177 (R2D2(C162V/Y221S/R222K)-R2D3(S283T)-Fc)
SPFIASVSDQHGVVYITENKNKTVVIPCLGSISNLNVSLVARYPEKRFVPDGNRISWDSKKGFTIPSYMISYAGMVFCEAKINDESYQSIMYIVVVVGSKIYDVVLSPSHGIELSVGEKLVLNCTARTELNVGIDFNWEYPSSKHQHKKLVNRDLKTQSGTEMKKFLSTLTIDGVTRSDQGLYTCAASSGLMTKKNSTFVRVHEKDKTHTCPPCPAPEAAGGPSVFLFPPKPKDTLMISRTPEVTCVVVDVSHEDPEVKFNWYVDGVEVHNAKTKPREEQYNSTYRVVSVLTVLHQDWLNGKEYKCKVSNKALPAPIEKTISKAKGQPREPQVYTLPPSREEMTKNQVSLTCLVKGFYPSDIAVEWESNGQPENNYKTTPPVLDSDGSFFLYSKLTVDKSRWQQGNVFSCSVMHEALHNHYTQKSLSLSPGK

SEQ ID NO: 65 - protein, 432 aa, synthetic construct
  source 1..432: note = PR1178 (R2D2(C162V/Y221S/R222K)-R2D3(N274F/S283T)-Fc)
SPFIASVSDQHGVVYITENKNKTVVIPCLGSISNLNVSLVARYPEKRFVPDGNRISWDSKKGFTIPSYMISYAGMVFCEAKINDESYQSIMYIVVVVGSKIYDVVLSPSHGIELSVGEKLVLNCTARTELNVGIDFNWEYPSSKHQHKKLVFRDLKTQSGTEMKKFLSTLTIDGVTRSDQGLYTCAASSGLMTKKNSTFVRVHEKDKTHTCPPCPAPEAAGGPSVFLFPPKPKDTLMISRTPEVTCVVVDVSHEDPEVKFNWYVDGVEVHNAKTKPREEQYNSTYRVVSVLTVLHQDWLNGKEYKCKVSNKALPAPIEKTISKAKGQPREPQVYTLPPSREEMTKNQVSLTCLVKGFYPSDIAVEWESNGQPENNYKTTPPVLDSDGSFFLYSKLTVDKSRWQQGNVFSCSVMHEALHNHYTQKSLSLSPGK

SEQ ID NO: 66 - protein, 637 aa, synthetic construct
  source 1..637: note = PR1179 (R1D2-R2D3-R2D2(C162V/Y221S/R222K)-R2D3-Fc)
SDTGRPFVEMYSEIPEIIHMTEGRELVIPCRVTSPNITVTLKKFPLDTLIPDGKRIIWDSRKGFIISNATYKEIGLLTCEATVNGHLYKTNYLTHRQTNTIIDVVLSPSHGIELSVGEKLVLNCTARTELNVGIDFNWEYPSSKHQHKKLVNRDLKTQSGSEMKKFLSTLTIDGVTRSDQGLYTCAASSGLMTKKNSTFVRVHEKSPFIASVSDQHGVVYITENKNKTVVIPCLGSISNLNVSLVARYPEKRFVPDGNRISWDSKKGFTIPSYMISYAGMVFCEAKINDESYQSIMYIVVVVGSKIYDVVLSPSHGIELSVGEKLVLNCTARTELNVGIDFNWEYPSSKHQHKKLVNRDLKTQSGSEMKKFLSTLTIDGVTRSDQGLYTCAASSGLMTKKNSTFVRVHEKDKTHTCPPCPAPEAAGGPSVFLFPPKPKDTLMISRTPEVTCVVVDVSHEDPEVKFNWYVDGVEVHNAKTKPREEQYNSTYRVVSVLTVLHQDWLNGKEYKCKVSNKALPAPIEKTISKAKGQPREPQVYTLPPSREEMTKNQVSLTCLVKGFYPSDIAVEWESNGQPENNYKTTPPVLDSDGSFFLYSKLTVDKSRWQQGNVFSCSVMHEALHNHYTQKSLSLSPGK

SEQ ID NO: 67 - protein, 677 aa, synthetic construct
  source 1..677: note = PR1186 (heavy chain H: R1D2-R2D3-R2D2(C162V/Y221S/R222K)-R2D3(N274F/S283T)-Fc-linker-VH-CH1)
SPFIASVSDQHGVVYITENKNKTVVIPCLGSISNLNVSLVARYPEKRFVPDGNRISWDSKKGFTIPSYMISYAGMVFCEAKINDESYQSIMYIVVVVGSKIYDVVLSPSHGIELSVGEKLVLNCTARTELNVGIDFNWEYPSSKHQHKKLVFRDLKTQSGTEMKKFLSTLTIDGVTRSDQGLYTCAASSGLMTKKNSTFVRVHEKDKTHTCPPCPAPEAAGGPSVFLFPPKPKDTLMISRTPEVTCVVVDVSHEDPEVKFNWYVDGVEVHNAKTKPREEQYNSTYRVVSVLTVLHQDWLNGKEYKCKVSNKALPAPIEKTISKAKGQPREPQVYTLPPSREEMTKNQVSLTCLVKGFYPSDIAVEWESNGQPENNYKTTPPVLDSDGSFFLYSKLTVDKSRWQQGNVFSCSVMHEALHNHYTQKSLSLSPGGGGGSGGGGSGGGGSGGGGSEVQLVESGGGLVQPGGSLRLSCAASGYTFTNYGMNWVRQAPGKGLEWVGWINTYTGEPTYAADFKRRFTFSLDTSKSTAYLQMNSLRAEDTAVYYCAKYPHYYGSSHWYFDVWGQGTLVTVSSASTKGPSVFPLAPSSKSTSGGTAALGCLVKDYFPEPVTVSWNSGALTSGVHTFPAVLQSSGLYSLSSVVTVPSSSLGTQTYICNVNHKPSNTKVDKKVEPKSC

SEQ ID NO: 68 - protein, 214 aa, synthetic construct; identical to SEQ ID NO: 51
  source 1..214: note = PR1186 light chain L: VL-CL

SEQ ID NO: 69 - protein, 205 aa, Homo sapiens
  source 1..205: note = Wild-type VEGFR2 D2D3
SPFIASVSDQHGVVYITENKNKTVVIPCLGSISNLNVSLCARYPEKRFVPDGNRISWDSKKGFTIPSYMISYAGMVFCEAKINDESYQSIMYIVVVVGYRIYDVVLSPSHGIELSVGEKLVLNCTARTELNVGIDFNWEYPSSKHQHKKLVNRDLKTQSGSEMKKFLSTLTIDGVTRSDQGLYTCAASSGLMTKKNSTFVRVHEK

SEQ ID NO: 70 - protein, 431 aa, synthetic construct
  source 1..431: note = Aflibercept(PR1076)
SDTGRPFVEMYSEIPEIIHMTEGRELVIPCRVTSPNITVTLKKFPLDTLIPDGKRIIWDSRKGFIISNATYKEIGLLTCEATVNGHLYKTNYLTHRQTNTIIDVVLSPSHGIELSVGEKLVLNCTARTELNVGIDFNWEYPSSKHQHKKLVNRDLKTQSGSEMKKFLSTLTIDGVTRSDQGLYTCAASSGLMTKKNSTFVRVHEKDKTHTCPPCPAPELLGGPSVFLFPPKPKDTLMISRTPEVTCVVVDVSHEDPEVKFNWYVDGVEVHNAKTKPREEQYNSTYRVVSVLTVLHQDWLNGKEYKCKVSNKALPAPIEKTISKAKGQPREPQVYTLPPSRDELTKNQVSLTCLVKGFYPSDIAVEWESNGQPENNYKTTPPVLDSDGSFFLYSKLTVDKSRWQQGNVFSCSVMHEALHNHYTQKSLSLSPG

SEQ ID NO: 71 - protein, 537 aa, synthetic construct
  source 1..537: note = OPT-302(HRAMD-C3)
YSMTPPTLNITEESHVIDTGDSLSISCRGQHPLEWAWPGAQEAPATGDKDSEDTGVVRDCEGTDARPYCKVLLLHEVHAQDTGSYVCYYKYIKARIEGTTAASSYVFVRDFEQPFINKPDTLLVNRKDAMWVPCLVSIPGLNVTLRSQSSVLWPDGQEVVWDDRRGMLVSTPLLHDALYLQCETTWGDQDFLSNPFLVHITGNELYDIQLLPRKSLELLVGEKLVLNCTVWAEFNSGVTFDWDYPGKQAERGKWVPERRSQQTHTELSSILTIHNVSQHDLGSYVCKANNGIQRFRESTEVIVHEEPKSCDKTHTCPPCPAPELLGGPSVFLFPPKPKDTLMISRTPEVTCVVVDVSHEDPEVKFNWYVDGVEVHNAKTKPREEQYNSTYRVVSVLTVLHQDWLNGKEYKCKVSNKALPAPIEKTISKAKGQPREPQVYTLPPSRDELTKNQVSLTCLVKGFYPSDIAVEWESNGQPENNYKTTPPVLDSDGSFFLYSKLTVDKSRWQQGNVFSCSVMHEALHNHYTQKSLSLSPGK

SEQ ID NO: 72 - protein, 453 aa, synthetic construct
  source 1..453: note = Bevacizumab heavy chain
EVQLVESGGGLVQPGGSLRLSCAASGYTFTNYGMNWVRQAPGKGLEWVGWINTYTGEPTYAADFKRRFTFSLDTSKSTAYLQMNSLRAEDTAVYYCAKYPHYYGSSHWYFDVWGQGTLVTVSSASTKGPSVFPLAPSSKSTSGGTAALGCLVKDYFPEPVTVSWNSGALTSGVHTFPAVLQSSGLYSLSSVVTVPSSSLGTQTYICNVNHKPSNTKVDKKVEPKSCDKTHTCPPCPAPEAAGGPSVFLFPPKPKDTLMISRTPEVTCVVVDVSHEDPEVKFNWYVDGVEVHNAKTKPREEQYNSTYRVVSVLTVLHQDWLNGKEYKCKVSNKALPAPIEKTISKAKGQPREPQVYTLPPSREEMTKNQVSLTCLVKGFYPSDIAVEWESNGQPENNYKTTPPVLDSDGSFFLYSKLTVDKSRWQQGNVFSCSVMHEALHNHYTQKSLSLSPGK

SEQ ID NO: 73 - protein, 214 aa, synthetic construct; identical to SEQ ID NO: 51
  source 1..214: note = Bevacizumab light chain

SEQ ID NO: 74 - DNA, 304 bp, synthetic construct
  source 1..304: mol_type = other DNA; note = CMV enhancer sequence
cgttacataacttacggtaaatggcccgcctggctgaccgcccaacgacccccgcccattgacgtcaataatgacgtatgttcccatagtaacgccaatagggactttccattgacgtcaatgggtggagtatttacggtaaactgcccacttggcagtacatcaagtgtatcatatgccaagtacgccccctattgacgtcaatgacggtaaatggcccgcctggcattatgcccagtacatgaccttatgggactttcctacttggcagtacatctacgtattagtcatcgctattaccatg

SEQ ID NO: 75 - DNA, 309 bp, synthetic construct
  source 1..309: mol_type = other DNA; note = CMV promoter sequence
tgctgatgcggttttggcagtacaccaatgggcgtggatagcggtttgactcacggggatttccaagtctccaccccattgacgtcaatgggagtttgttttggcaccaaaatcaacgggactttccaaaatgtcgtaataaccccgccccgttgacgcaaatgggcggtaggcgtgtacggtgggaggtctatataagcagagctcgtttagtgaaccgtcagatcgcctggagaggccatccacgctgttttgacctccatagtggacaccgggaccgatccagcctccgcgtctcaggggaagctt

SEQ ID NO: 76 - DNA, 43 bp, synthetic construct
  source 1..43: mol_type = other DNA; note = 5'UTR sequence
cttgttctttttgcagaagctcagaataaacgctcaactttgg

SEQ ID NO: 77 - protein, 745 aa, synthetic construct
  source 1..745: note = Capsid protein
MAADGYLPDWLEDTLSEGIRQWWKLKPGPPPPKPAERHKDDSRGLVLPGYKYLGPFNGLDKGEPVNEADAAALEHDKAYDRQLDSGDNPYLKYNHADAEFQERLKEDTSFGGNLGRAVFQAKKRVLEPLGLVEEPVKTAPGKKRPVEHSPVEPDSSSGTGKAGQQPARKRLNFGQTGDADSVPDPQPLGQPPAAPSGLGTNTMATGSGAPMADNNEGADGVGNSSGNWHCDSTWMGDRVITTSTRTWALPTYNNHLYKQISSQSGASNDNHYFGYSTPWGYFDFNRFHCHFSPRDWQRLINNNWGFRPKRLNFKLFNIQVKEVTQNDGTTTIANNLTSTVQVFTDSEYQLPYVLGSAHQGCLPPFPADVFMVPQYGYLTLNNGSQAVGRSSFYCLEYFPSQMLRTGNNFTFSYTFEDVPFHSSYAHSQSLDRLMNPLIDQYLYYLSRTNTPSGTTTQSRLQFSQAGASDIRDQSRNWLPGPCYRQQRVSKTSADNNNSEYSWTGATKYHLNGRDSLVNPGPAMASHKDDEEKFFPQSGVLIFGKQGSEKTNVDIEKVMITDEEEIRTTNPVATEQYGSVSTNLQRGNLALGDTTRPARQAATADVNTQGVLPGMVWQDRDVYLQGPIWAKIPHTDGHFHPSPLMGGFGLKHPPPQILIKNTPVPANPSTTFSAAKFASFITQYSTGQVSVEIEWELQKENSKRWNPEIQYTSNYNKSINVDFTVDTNGVYSEPRPIGTRYLTRNL

SEQ ID NO: 78 - DNA, 1977 bp, synthetic construct
  source 1..1977: mol_type = other DNA; note = Codon-optimized sequence 1 of PR1145
atgcctctgctgctgctgttgcctttgttgtgggctggcgccctggcttctgataccggcagacctttcgtggaaatgtacagcgagatccccgagatcatccacatgaccgagggcagagagctggtcatcccctgcagagtgacctctcctaacatcaccgtgactctgaagaagttccctctggacacactgatccccgacggcaagagaatcatctgggactcccggaagggcttcatcatctccaacgccacctacaaagagatcggcctgctgacctgcgaggccaccgttaatggccacctgtacaagaccaactatctgacccacagacagaccaacaccatcatcgacgtggtgctgagcccctctcatggcatcgagctgtccgtgggagaaaagctggtgctgaactgcaccgccagaaccgagctgaacgtgggcatcgacttcaactgggagtacccctccagcaagcaccagcacaagaagctggtcaaccgggacctgaaaacccagtccggctccgagatgaagaaattcctgagcaccctgaccatcgacggcgtgaccagatctgaccagggcctgtatacctgcgccgcttcttctggcctgatgaccaagaaaaactccaccttcgtgcgggtgcacgagaaaggtggcggaggcagctctccttttatcgcctctgtgtctgatcagcacggcgtggtgtacatcaccgagaacaagaacaagaccgtcgtgatcccctgcctgggctccatctctaacctgaacgtgtccctggtggctagataccccgagaagagattcgtgcctgacggcaaccggatctcctgggacagcaagaagggctttacaatcccctcctacatgatctcctacgccggcatggtgttctgcgaggctaagatcaacgacgagtcctaccagtccatcatgtacatcgtggtggtcgtgggctacagaatctacgatgtggtgctgtcccctagccacggaatcgaactgagcgtgggcgagaaactggtcctcaactgtaccgctcggacagaactgaatgtggggattgatttcaattgggaataccctagctccaaacatcagcataagaaactcgtgaaccgcgatctcaagacccagagcggaacagaaatgaagaagtttctgtccacactcaccattgacggggtcaccagaagcgatcagggactctatacctgtgctgcctccagcggactgatgacaaaaaagaacagcacatttgtccgcgtccacgagaaggacaaaactcacacatgcccaccgtgcccggcgcctgaagccgctgggggaccgtcagtcttcctcttccccccaaaacccaaggacaccctcatgatctcccggacccctgaggtcacatgcgtggtggtggacgtgagccacgaagaccctgaggtcaagttcaactggtacgtggacggcgtggaggtgcataatgccaagacaaagccgcgggaggagcagtacaacagcacgtaccgggtggtcagcgtcctcaccgtcctgcaccaggactggctgaatggcaaggagtacaagtgcaaggtctccaacaaagccctcccagcccccatcgagaaaaccatctccaaagccaaagggcagcccagggaaccacaggtgtacaccctgcccccatcccgggaggagatgaccaagaaccaggtcagcctgacctgcctggtcaaaggcttctatcccagcgacatcgccgtggagtgggagagcaatgggcagccggagaacaactacaagaccacgcctcccgtgctggactccgacggctccttcttcctctacagcaagctcaccgtggacaagagcaggtggcagcaggggaacgtcttctcatgctccgtgatgcatgaggctctgcacaaccactacacgcagaagagcctctccctgtctccgggtaaataa

SEQ ID NO: 79 - DNA, 1977 bp, synthetic construct
  source 1..1977: mol_type = other DNA; note = Codon-optimized sequence 2 of PR1145
atgcctctgctgctgctgctgcctctgctgtgggccggcgccctggcctccgacaccggccggccttttgttgaaatgtactccgagatccccgaaatcatccacatgacagaaggcagagagctggtgatcccttgtagagtgaccagcccaaacatcaccgtgactctgaagaagttccccctggatacactgatccctgatggaaagagaatcatttgggatagcagaaagggctttatcatcagcaacgccacatacaaagagatcggcctgctcacctgcgaggccaccgtgaacggccacctgtataagacaaactacctgacacatagacagaccaacaccatcattgacgtggtgctgtccccaagccacggaatcgagctgtctgtgggcgagaagctggtgctgaactgcaccgccagaacagagctgaacgtgggcattgacttcaattgggagtaccctagctccaaacaccaacacaagaagctggtgaatagagatctgaaaacccagtctggcagcgaaatgaagaaatttctgagcacactgaccattgacggcgtgacccgcagcgaccagggcctgtacacctgtgccgcctcttctggccttatgaccaaaaaaaattctaccttcgtgcgggtgcacgagaagggcggaggcggctctagccccttcatcgccagcgtcagcgatcagcacggcgtggtctacatcaccgaaaacaagaacaagaccgtggtcattccttgcctgggcagcatcagtaatctgaacgtgagcctggtggccagataccctgagaagcggttcgtgcccgacggcaacaggatcagctgggacagcaagaagggctttacgatcccctcttatatgatctcctacgccggaatggtgttctgcgaggctaagatcaacgacgagagctaccagagcatcatgtacatcgtggtcgtggtcggctaccggatctacgacgtggtgctgagcccttctcacggcatcgagctgtccgtcggagagaagctggtgttgaattgcaccgccagaaccgagctgaacgtgggcatcgactttaactgggaataccccagctctaaacaccagcacaagaagctggtgaaccgggacctgaagacccaatctggtacagagatgaagaagttcctaagcacactgaccatcgacggcgtcacaagaagcgatcagggactgtacacctgcgccgctagcagcggactgatgaccaagaaaaacagcaccttcgtgcgggtgcacgagaaagacaagacacacacctgccctccatgtcctgcccctgaagctgctggcggaccttctgtgttcctcttcccacctaagcctaaggacaccctgatgatcagccggacacctgaagtgacatgcgtggtggtggatgtgtctcacgaagatcccgaggtgaaattcaactggtacgtggacggcgttgaagtgcataatgccaagaccaagcccagagaggaacagtacaacagcacctacagagtggtgtccgtactgaccgtgctgcaccaggactggctgaacggcaaggaatacaagtgcaaggtgtccaacaaagccctgcctgcccctatcgagaagaccatctctaaggccaagggccagcctagagaaccccaagtgtacacactgcctccttccagagaggaaatgaccaagaaccaggtgtcattgacatgtctggtgaaggggttctacccaagcgacatcgccgtggaatgggagagcaacggacagcccgagaacaactacaagaccacacctccagtgctcgatagcgacggcagcttcttcctgtatagcaagctgaccgtggacaagtccagatggcagcagggcaatgtgttcagctgcagcgtgatgcacgaggctctgcacaaccactacacccagaagagcctgtccctgagccccggcaagtga

SEQ ID NO: 80 - DNA, 1977 bp, synthetic construct
  source 1..1977: mol_type = other DNA; note = Codon-optimized sequence 3 of PR1145
atgcccctgctcctgctcctgcccctgctgtgggccggcgccctggctagcgacaccggcagacccttcgtggagatgtacagcgagatccccgagatcatccacatgaccgagggcagagagctcgtgatcccttgcagagtgacaagccccaacatcaccgtgaccctgaaaaagttccccctggacaccctgatccccgacggcaagagaatcatctgggacagcagaaagggcttcatcatcagcaacgccacctacaaggagatcggcctgctgacctgcgaggccaccgtgaacggccacctgtacaagaccaactacctgacccacagacagaccaacaccatcatcgacgtcgtgctgagccctagccacggcatcgagctgagcgtgggcgaaaaactggtcctcaactgtaccgctcggaccgaactgaacgtggggatcgatttcaactgggagtatcctagctccaagcatcagcataagaagctggtcaacagagatctcaagacacagagcggctccgaaatgaaaaaattcctctccaccctgacaattgacggcgtcacacggagcgaccaaggcctgtatacctgcgctgctagcagcgggctgatgaccaagaagaactccacctttgtcagagtgcacgaaaagggcgggggcggcagcagccccttcatcgctagcgtgagcgatcagcacggcgtggtgtacatcaccgagaacaagaacaagaccgtggtgatcccctgcctgggcagcatcagcaacctgaacgtgagcctggtggctagataccccgagaagagattcgtgcccgacggcaacagaatcagctgggacagcaagaagggcttcaccatccctagctacatgatcagctacgccggcatggtgttctgcgaggccaagatcaacgacgagagctatcagagcatcatgtacatcgtggtcgtggtgggctacagaatctacgacgtggtgctgtcccctagccacggcattgaactgtccgtgggggagaagctggtgctgaactgtaccgcccggacagagctgaacgtgggcatcgactttaactgggagtaccctagcagcaaacatcagcacaagaagctggtgaaccgggacctgaagacacagagcggcacagaaatgaagaaattcctgagcacactgacaattgatggcgtgacaagaagcgaccaaggcctgtacacctgcgccgctagcagcggcctcatgacaaagaagaacagcacatttgtgcgggtgcacgagaaagacaaaacacatacctgtcctccctgtcccgcccctgaagccgctggggggcctagcgtgttcctgttcccccccaagcccaaggacacactgatgatcagcagaacccccgaggtgacctgcgtggtcgtggacgtgagccacgaggaccccgaggtgaagttcaactggtacgtggacggcgtggaggtgcacaacgccaagaccaagcctagagaggagcagtacaacagcacctacagagtggtgagcgtgctgaccgtgctgcaccaagactggctgaacggcaaggagtacaagtgcaaggtgagcaacaaggccctgcccgcccccatcgagaagaccatcagcaaggccaaggggcagcctagagagccccaagtgtacaccctgccccctagcagagaggagatgaccaaaaaccaagtgagcctgacctgcctggtgaagggcttctaccctagcgacatcgccgtggagtgggagagcaacgggcagcccgagaacaactacaagaccaccccccccgtgctggacagcgacggcagcttcttcctgtacagcaagctgaccgtggacaagagcagatggcagcaaggcaacgtgttcagctgcagcgtgatgcacgaggccctgcacaaccactacacacagaagagcctgagcctgagccccggcaagtga

SEQ ID NO: 81 - DNA, 1977 bp, synthetic construct
  source 1..1977: mol_type = other DNA; note = Codon-optimized sequence 1 of PR1174
atgcctctgctgctgctgttgcctttgttgtgggctggcgccctggcttctgataccggcagacctttcgtggaaatgtacagcgagatccccgagatcatccacatgaccgagggcagagagctggtcatcccctgcagagtgacctctcctaacatcaccgtgactctgaagaagttccctctggacacactgatccccgacggcaagagaatcatctgggactcccggaagggcttcatcatctccaacgccacctacaaagagatcggcctgctgacctgcgaggccaccgttaatggccacctgtacaagaccaactatctgacccacagacagaccaacaccatcatcgacgtggtgctgagcccctctcatggcatcgagctgtccgtgggagaaaagctggtgctgaactgcaccgccagaaccgagctgaacgtgggcatcgacttcaactgggagtacccctccagcaagcaccagcacaagaagctggtcaaccgggacctgaaaacccagtccggctccgagatgaagaaattcctgagcaccctgaccatcgacggcgtgaccagatctgaccagggcctgtatacctgcgccgcttcttctggcctgatgaccaagaaaaactccaccttcgtgcgggtgcacgagaaaggtggcggaggcagctctccttttatcgcctctgtgtctgatcagcacggcgtggtgtacatcaccgagaacaagaacaagaccgtcgtgatcccctgcctgggctccatctctaacctgaacgtgtccctggtggctagataccccgagaagagattcgtgcctgacggcaaccggatctcctgggacagcaagaagggctttacaatcccctcctacatgatctcctacgccggcatggtgttctgcgaggctaagatcaacgacgagtcctaccagtccatcatgtacatcgtggtggtcgtgggctccaagatctacgatgtggtgctgtcccctagccacggaatcgaactgagcgtgggcgagaaactggtcctcaactgtaccgctcggacagaactgaatgtggggattgatttcaattgggaataccctagctccaaacatcagcataagaaactcgtgttccgcgatctcaagacccagagcggaacagaaatgaagaagtttctgtccacactcaccattgacggggtcaccagaagcgatcagggactctatacctgtgctgcctccagcggactgatgacaaaaaagaacagcacatttgtccgcgtccacgagaaggacaaaactcacacatgcccaccgtgcccggcgcctgaagccgctgggggaccgtcagtcttcctcttccccccaaaacccaaggacaccctcatgatctcccggacccctgaggtcacatgcgtggtggtggacgtgagccacgaagaccctgaggtcaagttcaactggtacgtggacggcgtggaggtgcataatgccaagacaaagccgcgggaggagcagtacaacagcacgtaccgggtggtcagcgtcctcaccgtcctgcaccaggactggctgaatggcaaggagtacaagtgcaaggtctccaacaaagccctcccagcccccatcgagaaaaccatctccaaagccaaagggcagcccagggaaccacaggtgtacaccctgcccccatcccgggaggagatgaccaagaaccaggtcagcctgacctgcctggtcaaaggcttctatcccagcgacatcgccgtggagtgggagagcaatgggcagccggagaacaactacaagaccacgcctcccgtgctggactccgacggctccttcttcctctacagcaagctcaccgtggacaagagcaggtggcagcaggggaacgtcttctcatgctccgtgatgcatgaggctctgcacaaccactacacgcagaagagcctctccctgtctccgggtaaataa

SEQ ID NO: 82 - DNA, 1977 bp, synthetic construct
  source 1..1977: mol_type = other DNA; note = Codon-optimized sequence 2 of PR1174
atgcctctgctgctgctcctgcctctgctgtgggccggcgccctggccagcgataccggcagaccattcgtggaaatgtacagcgaaatccccgagatcatccacatgaccgagggcagagaactggtgatcccctgcagagtgaccagcccaaacatcaccgtgaccctcaagaagtttcccctggacaccctgatccctgatggaaaaagaatcatctgggacagcagaaagggctttatcatttctaatgccacatacaaagagataggactgttgacctgtgaagctacagttaacggccacctgtacaagaccaactacctgacccaccggcagacaaacaccatcatcgacgtggtgctgagccctagccacggaatcgagctgtccgtgggagaaaagctggtgctgaattgcaccgccagaaccgagctgaacgtaggcatcgacttcaactgggagtatccttcaagcaaacatcagcacaaaaaactggtgaacagagacctgaagacccagagtggcagcgagatgaaaaagttcctgagcacactgacaatcgacggagtgactcggagcgatcagggcctgtatacatgtgctgcttctagcggcctgatgacaaagaagaacagcacattcgtgcgggtgcacgagaaggggggcggcggatcttccccattcatcgccagcgtgtccgaccagcatggcgtggtttacatcacagaaaacaagaacaagaccgtggtgatcccctgcctgggctccatcagcaacctgaatgtgtcgctggtggccagataccccgaaaagcggttcgtccccgacggcaacagaatcagctgggacagcaaaaagggcttcaccatcccaagctatatgatcagctacgccggaatggtgttctgcgaggccaaaatcaacgacgagtcctaccagagcatcatgtacatcgtggtggttgtcggcagcaagatctacgacgtcgtgctgagcccatctcacggcattgagctgtctgtgggcgagaagctggtgctgaattgcaccgcccggacagaactcaatgtgggcatcgatttcaactgggagtaccctagctctaagcaccagcacaagaagctggtctttagagatctgaaaacccaatctggcaccgagatgaaaaagttcctgagcaccctgaccatcgacggcgtgaccagaagcgaccagggcctgtacacctgcgccgcctctagcggcctgatgaccaagaaaaacagcaccttcgtgcgcgttcacgagaaagataagacacacacctgtcctccttgtcctgcccctgaggccgctggcggaccttctgtgttcctgttccctccaaagcccaaggacaccctgatgatcagcagaacacccgaagtgacctgcgtggtggtggacgtctctcacgaggaccccgaggtgaaatttaactggtacgtggacggcgtcgaggtgcataatgccaagacaaagcctcgggaagagcagtacaacagcacatacagagtggtcagcgtgctgacagtgctgcaccaggattggctgaacggcaaggaatacaagtgcaaggtgagcaacaaggccctgcctgctcctatcgagaagaccattagcaaggccaagggccagcctagggagcctcaggtgtacaccttaccacctagcagagaggaaatgacgaagaaccaggtgtccctgacatgcctggtgaagggtttctacccttctgatatcgccgtggaatgggaatccaacggccaacctgagaacaactacaagaccacccctcccgtgctcgatagcgacggctccttcttcctgtacagcaagctgaccgtggataagagccggtggcagcagggcaatgtgtttagctgctctgtgatgcacgaagccctgcacaaccactacacccaaaagagcctgagcctgagccccggcaagtga

SEQ ID NO: 83 - DNA, 1977 bp, synthetic construct
  source 1..1977: mol_type = other DNA; note = Codon-optimized sequence 3 of PR1174
atgcccctgctcctgctcctgcccctgctgtgggccggcgccctggctagcgacaccggcagacccttcgtggagatgtacagcgagatccccgagatcatccacatgaccgagggcagagagctcgtgatcccttgcagagtgacaagccccaacatcaccgtgaccctgaaaaagttccccctggacaccctgatccccgacggcaagagaatcatctgggacagcagaaagggcttcatcatcagcaacgccacctacaaggagatcggcctgctgacctgcgaggccaccgtgaacggccacctgtacaagaccaactacctgacccacagacagaccaacaccatcatcgacgtcgtgctgagccctagccacggcatcgagctgtccgtgggcgaaaagctcgtcctgaactgcaccgctagaaccgaactcaacgtggggattgatttcaactgggagtatcctagctccaagcaccaacacaagaagctggtgaaccgggatctgaagacacagagcgggagcgagatgaagaagttcctgagcaccctgacaatcgacggggtgacaagatccgaccaaggcctgtacacctgcgctgctagcagcggcctgatgacaaagaaaaatagcacatttgtgagagtgcacgagaagggcgggggcggcagcagccccttcatcgctagcgtgagcgatcagcacggcgtggtgtacatcaccgagaacaagaacaagaccgtggtgatcccctgcctgggcagcatcagcaacctgaacgtgagcctggtggctagataccccgagaagagattcgtgcccgacggcaacagaatcagctgggacagcaagaagggcttcaccatccctagctacatgatcagctacgccggcatggtgttctgcgaggccaagatcaacgacgagagctatcagagcatcatgtacatcgtggtcgtggtgggcagcaagatctacgacgtggtgctgagcccctcccacggcattgagctcagcgtgggcgagaagctggtcctcaactgcacagcccggaccgagctgaacgtgggcatcgattttaactgggagtaccctagcagcaagcatcagcataaaaagctggtgttccgggacctgaagacccaaagcggcaccgaaatgaagaagtttctctccaccctgaccatcgacggcgtgacaagaagcgaccaaggcctgtacacatgcgccgctagctccggcctcatgacaaagaagaattccacctttgtcagagtccatgaaaaagataagacacacacctgtcccccttgtcccgcccccgaagccgctgggggccctagcgtgttcctgttcccccccaagcccaaggataccctgatgatcagcagaacccccgaggtgacctgcgtggtcgtggacgtgagccacgaggaccccgaggtgaagttcaactggtacgtggacggcgtggaggtgcacaacgccaagaccaagcctagagaggagcagtacaacagcacctacagagtggtgagcgtgctgaccgtgctgcaccaagactggctgaacggcaaggagtacaagtgcaaggtgagcaacaaggccctgcccgcccccatcgagaagaccatcagcaaggccaaggggcagcctagagagccccaagtgtacaccctgccccctagcagagaggagatgaccaagaaccaagtgagcctgacctgcctggtgaagggcttctaccctagcgacatcgccgtggagtgggagagcaacgggcagcccgagaacaactacaagaccaccccccccgtgctggacagcgacggcagcttcttcctgtacagcaagctgaccgtggacaagagcagatggcagcaaggcaacgtgttcagctgcagcgtgatgcacgaggccctgcacaaccactacacacagaagagcctgagcctgagccccggcaagtga

SEQ ID NO: 84 - DNA, 2826 bp, synthetic construct
  source 1..2826: mol_type = other DNA; note = Codon-optimized sequence 1 of PR1163
atgcctctgctgctgctgttgcctttgttgtgggctggcgctctggcctctccttttatcgcctctgtgtctgatcagcacggcgtggtgtacatcaccgagaacaagaacaagaccgtcgtgatcccctgcctgggctccatctctaacctgaacgtgtccctggtggctagataccccgagaagagattcgtgcctgacggcaaccggatctcctgggacagcaagaagggctttacaatcccctcctacatgatctcctacgccggcatggtgttctgcgaggctaagatcaacgacgagtcctaccagtccatcatgtacatcgtggtggtcgtgggctacagaatctacgatgtggtgctgtcccctagccacggaatcgaactgagcgtgggcgagaaactggtcctcaactgtaccgctcggacagaactgaatgtggggattgatttcaattgggaataccctagctccaaacatcagcataagaaactcgtgaaccgcgatctcaagacccagagcggaagcgaaatgaagaagtttctgtccacactcaccattgacggggtcaccagaagcgatcagggactctatacctgtgctgcctccagcggactgatgacaaaaaagaacagcacatttgtccgcgtccacgagaaggacaaaactcacacatgcccaccgtgcccggcgcctgaagccgctgggggaccgtcagtcttcctcttccccccaaaacccaaggacaccctcatgatctcccggacccctgaggtcacatgcgtggtggtggacgtgagccacgaagaccctgaggtcaagttcaactggtacgtggacggcgtggaggtgcataatgccaagacaaagccgcgggaggagcagtacaacagcacgtaccgggtggtcagcgtcctcaccgtcctgcaccaggactggctgaatggcaaggagtacaagtgcaaggtctccaacaaagccctcccagcccccatcgagaaaaccatctccaaagccaaagggcagcccagggaaccacaggtgtacaccctgcccccatcccgggaggagatgaccaagaaccaggtcagcctgacctgcctggtcaaaggcttctatcccagcgacatcgccgtggagtgggagagcaatgggcagccggagaacaactacaagaccacgcctcccgtgctggactccgacggctccttcttcctctacagcaagctcaccgtggacaagagcaggtggcagcaggggaacgtcttctcatgctccgtgatgcatgaggctctgcacaaccactacacgcagaagagcctctccctgtctccgggtggcggaggcggctccggtggaggcggttcaggcggaggtggctctggcggtggcggatcggaggtgcagctggtggagagcggggggggactggtgcagccaggaggaagcctgagactgagctgtgccgccagcgggtacacatttaccaactacggaatgaactgggtgaggcaggctcctggcaaggggctggagtgggtggggtggattaacacctacaccggagagcccacatacgctgctgattttaagcggagattcaccttcagcctggacaccagcaagagcaccgcttacctgcagatgaacagcctgagagccgaggacacagccgtgtactactgcgccaaatacccccattactacggcagcagccactggtacttcgacgtgtggggccagggaacactggtgaccgtgagcagcgctagcaccaagggcccatcggtcttccccctggcaccctcctccaagagcacctctgggggcacagcggccctgggctgcctggtcaaggactacttccccgaaccggtgacggtgtcgtggaactcaggcgccctgaccagcggcgtgcacaccttcccggctgtcctacagtcctcaggactctactccctcagcagcgtggtgaccgtgccctccagcagcttgggcacccagacctacatctgcaacgtgaatcacaagcccagcaacaccaaggtggacaagaaagttgagcccaaatcttgtgagggcagaggaagtcttctaacatgcggtgacgtggaggagaatcccggccctatgcctctgctgctgctgttgcctttgttgtgggctggcgctctggccgacattcagatgacccagagccccagcagcctgagcgccagcgtgggagacagagtgaccatcacctgcagcgccagccaggacatcagcaactacctgaactggtatcagcagaaacccggcaaagcccccaaagtgctgatctacttcacaagttcactgcacagcggagtgcccagcagattttcaggaagcggcagcggcaccgacttcaccctgaccatcagcagcctgcagcccgaggatttcgccacctactactgccagcagtactctaccgtgccatggaccttcggccaggggaccaaggtggaaatcaagcgtacggtggctgcaccatctgtcttcatcttcccgccatctgatgagcagttgaaatctggaactgcctctgttgtgtgcctgctgaataacttctatcccagagaggccaaagtacagtggaaggtggataacgccctccaatcgggtaactcccaggagagtgtcacagagcaggacagcaaggacagcacctacagcctcagcagcaccctgacgctgagcaaagcagactacgagaaacacaaagtctacgcctgcgaagtcacccatcagggcctgagttcgcccgtcacaaagagcttcaacaggggagagtgttaa

SEQ ID NO: 85 - DNA, 2826 bp, synthetic construct
  source 1..2826: mol_type = other DNA; note = Codon-optimized sequence 2 of PR1163
atgcctctgcttctgctgctgcctctgctttgggctggcgccctggccagccccttcatcgcctctgttagtgaccagcatggcgtggtgtatatcacggagaacaagaataagacagtagtgattccttgcctgggcagcatctctaatctgaacgtgtcgctggttgccagataccctgagaagagattcgtgcccgacggcaaccggatcagctgggacagcaagaagggctttaccatcccctcttacatgatcagctatgccggaatggtgttctgcgaagccaagatcaacgacgagtcctatcagtctatcatgtacatcgtggtcgtagtgggctacagaatctacgacgtggtgctgagcccatctcacggcatcgagctgagcgtgggagagaagctggtgctgaactgcacagctagaaccgagctgaacgtgggcatagacttcaactgggagtacccctccagcaagcaccagcacaagaaactggtcaacagagatctgaagacccagagcggctctgagatgaagaagttcctgtccaccctgacaatcgacggcgtgaccagaagcgatcagggactgtacacttgtgctgcgagctctggcctgatgaccaagaaaaacagcaccttcgtgcgggtgcacgagaaggacaagacccacacatgccctccttgtcctgcccctgaggccgctggcggccctagcgtgttcctgttcccccctaaacccaaggacaccctcatgatctcccggacacctgaagtgacttgcgtggtcgtggacgtcagccacgaagatccagaggtgaagttcaactggtatgtggatggcgtggaagtgcataatgcgaagacaaagcctcgggaagagcagtacaactccacgtacagagtggtgagcgtgctgaccgtgctgcatcaagactggctgaacggcaaggaatacaagtgcaaggtgtccaacaaggccctgcccgctcctatcgaaaaaaccatctctaaggccaagggccagcctagagagcctcaggtgtataccctgcctcctagccgggaagaaatgacaaagaaccaggtgtctctgacctgcctggtgaagggcttctaccccagcgacatcgccgtggagtgggagtccaacggccaacctgaaaacaattacaagaccacccctcccgtgctggacagcgacggcagcttcttcctgtattccaagctgaccgtcgacaagagcagatggcagcagggcaacgtgtttagctgtagcgtgatgcacgaggccctgcacaaccactacacacaaaagtctctgtccctgagccctggaggcggcggcggaagcggagggggcggctccggcggcggaggcagcggcggcggcggttccgaagtgcagctggtggaaagcggaggcggtctggttcagccgggcggcagcctgagactgtcttgcgccgccagcggctacacattcaccaactacggcatgaactgggtcagacaggcccctggcaagggcctggaatgggtgggatggatcaacacctacaccggcgaaccaacatacgccgctgattttaagcggaggttcaccttttctctggatacctccaaaagcaccgcctacctgcaaatgaacagcctgcgggccgaggacaccgccgtttactactgcgccaaatatcctcactactacggcagctctcactggtacttcgacgtttggggccagggcacactggtgaccgtgtcctcggccagcacaaagggccctagcgtgttcccactggcaccatctagcaagagcaccagtggaggcaccgccgccctgggatgcctggtgaaagattacttccccgagcctgtcaccgtgtcttggaactccggtgctctgacgagcggagtgcacaccttcccagccgtgcttcagtccagcggtctgtacagcctgtcttctgttgtgaccgtgccttccagctccctgggcacgcagacctacatctgcaacgtgaaccacaagcctagcaataccaaggtggataagaaggtggaacccaaaagctgcgagggaagaggctccctcctgacatgcggcgacgtggaagagaaccccggccctatgcccctgctgctgctgctgcctctgctgtgggccggcgccctggccgatatccagatgacccagtctccttcctccttatccgcctctgtgggcgacagagtgaccatcacctgttctgccagccaggatatcagcaactacctgaactggtaccagcagaagcccggcaaagccccaaaggtgctgatttacttcacaagcagcctgcacagcggagtgcctagccgcttcagcggctctggcagcgggaccgactttacactgaccattagcagcctgcagcctgaggatttcgccacatactactgtcagcaatacagcacagtcccttggacctttggacaaggaacaaaggtggaaatcaagcggaccgtggccgctcccagcgtgttcatcttccctcctagcgacgagcaactgaaatctggcaccgccagcgtcgtgtgcctgctgaacaacttctacccgagagaggctaaggtgcagtggaaggtggacaacgccctgcagagcgggaatagccaggagagcgtgaccgagcaggactccaaagacagcacatactctctgagcagcacccttacactgagcaaggccgactacgagaaacacaaagtgtacgcttgtgaggtgacccaccagggcctgagctctcccgtgaccaaaagctttaatagaggcgagtgctga

SEQ ID NO: 86 - DNA, 2826 bp, synthetic construct
  source 1..2826: mol_type = other DNA; note = Codon-optimized sequence 3 of PR1163
atgcctctgctgctgcttctgcctcttctttgggctggcgctctggctagcccttttatcgcctccgtgtccgatcagcacggcgtggtgtacatcaccgagaacaagaacaagaccgtggtcatcccctgcctgggcagcatcagcaacctgaatgtgtccctggtggccagatatcccgagaagagattcgtgcccgacggcaacagaatcagctgggacagcaagaagggcttcacaatccccagctacatgatcagctacgccggcatggtgttctgcgaggccaagatcaacgacgagagctaccagagcatcatgtacatcgtggtggtcgtgggctacagaatctacgacgtggtgctgagccctagccacggcattgaactgtctgtgggcgagaagctggtgctgaactgtaccgccagaaccgagctgaacgtgggcatcgacttcaactgggagtaccccagcagcaagcaccagcacaagaaactggtcaaccgggacctgaaaacccagagcggcagcgagatgaagaagttcctgagcaccctgaccatcgacggcgtgaccagatctgaccagggcctgtacacatgtgccgccagctctggcctgatgaccaagaaaaacagcaccttcgtgcgggtgcacgagaaggacaagacccacacctgtcctccatgtcctgctccagaagctgctggcggcccttccgtgtttctgttccctccaaagcctaaggacaccctgatgatcagcagaacccctgaagtgacctgcgtggtggtggatgtgtcccacgaggatcccgaagtgaagttcaattggtacgtggacggcgtggaagtgcacaacgccaagaccaagcctagagaggaacagtacaactccacctacagagtggtgtccgtgctgaccgtgctgcaccaggattggctgaacggcaaagagtacaagtgcaaggtgtccaacaaggccctgcctgctcctatcgagaaaaccatcagcaaggccaagggccagcctagggaaccccaggtttacacactgcctccaagccgggaagagatgacaaagaaccaggtgtccctgacctgcctggtcaagggcttctacccttccgatatcgccgtggaatgggagagcaatggccagcctgagaacaactacaagacaacccctcctgtgctggacagcgacggctcattcttcctgtacagcaagctgacagtggacaagagcagatggcagcagggcaacgtgttcagctgcagcgtgatgcacgaggccctgcacaaccactacacccagaagtccctgtctctgtctcctggcggaggcggaggatctggtggcggaggaagcggtggcggcggatcaggcggtggtggttctgaagttcagctggtggaaagcggcggtggccttgttcaacctggcggatctctgagactgagctgtgccgcctctggctacaccttcaccaactacggcatgaattgggtccgacaggcccctggcaaaggcctggaatgggtcggatggatcaacacctacaccggcgagccaacatacgccgccgacttcaagcggagattcaccttcagcctggacaccagcaagagcaccgcctacctgcagatgaactccctgagagccgaggacaccgccgtgtactactgcgccaagtatccccactactacggcagcagccactggtactttgacgtgtggggacagggcaccctggtcacagttagcagcgcctctacaaagggccccagcgttttcccactggctcctagcagcaagtctacctccggtggaacagctgccctgggctgtctcgtgaaggactactttcctgagcctgtgaccgtgtcctggaactctggcgcactgacatctggcgtgcacacctttccagctgtgctgcagtctagcggcctgtactctctgagcagcgtcgtgacagtgcctagcagctctctgggcacccagacctacatctgcaatgtgaaccacaagcctagcaacaccaaggtcgacaagaaggtggaacccaagagctgcgaaggcagaggcagcctgcttacatgtggcgacgtggaagagaaccccggacctatgccacttctcctgctgttgccattgctgtgggcaggcgcactggccgacattcagatgacacagagcccaagcagcctgagcgcctctgtgggagatagagtgaccatcacctgttccgccagccaggacatctccaactacctgaactggtatcagcaaaagcccggcaaggcccctaaggtgctgatctactttaccagcagcctgcacagcggcgtgcccagcagattttctggctctggcagcggcaccgacttcaccctgacaatatctagcctgcagccagaggacttcgccacctactactgccagcagtacagcaccgtgccttggacatttggccagggcaccaaggtggaaatcaagcggacagtcgccgctcctagcgtgttcatctttccacctagcgacgagcagctgaagtctggcacagcctctgtcgtgtgcctgctgaacaacttctaccccagagaagccaaggtgcagtggaaggtggacaatgccctgcagtccggcaacagccaagagagcgtgacagagcaggactccaaggacagcacctacagcctgtctagcacactgaccctgagcaaggccgactatgagaagcacaaagtgtacgcctgcgaagtgacccaccaggggctttctagcccagtgaccaagagcttcaaccggggcgagtgttga

SEQ ID NO: 87 - DNA, 133 bp, synthetic construct
  source 1..133: mol_type = other DNA; note = 3'-UTR sequence
gtctagaaaccagcctcaagaacacccgaatggagtctctaagctacataataccaacttacactttacaaaatgttgtcccccaaaatgtagccattcgtatctgctcctaataaaaagaaagtttcttcac

SEQ ID NO: 88 - DNA, 589 bp, synthetic construct
  source 1..589: mol_type = other DNA; note = WPRE sequence
aatcaacctctggattacaaaatttgtgaaagattgactggtattcttaactatgttgctccttttacgctatgtggatacgctgctttaatgcctttgtatcatgctattgcttcccgtatggctttcattttctcctccttgtataaatcctggttgctgtctctttatgaggagttgtggcccgttgtcaggcaacgtggcgtggtgtgcactgtgtttgctgacgcaacccccactggttggggcattgccaccacctgtcagctcctttccgggactttcgctttccccctccctattgccacggcggaactcatcgccgcctgccttgcccgctgctggacaggggctcggctgttgggcactgacaattccgtggtgttgtcggggaaatcatcgtcctttccttggctgctcgcctgtgttgccacctggattctgcgcgggacgtccttctgctacgtcccttcggccctcaatccagcggaccttccttcccgcggcctgctgccggctctgcggcctcttccgcgtcttcgccttcgccctcagacgagtcggatctccctttgggccgcctccccgc

SEQ ID NO: 89 - DNA, 140 bp, synthetic construct
  source 1..140: mol_type = other DNA; note = SV40polyA sequence
cctaggtaagatacattgatgagtttggacaaaccacaactagaatgcagtgaaaaaaatgctttatttgtgaaatttgtgatgctattgctttatttgtaaccattataagctgcaataaacaagttatcgatagatct

SEQ ID NO: 90 - protein, 15 aa, synthetic construct
  source 1..15: note = Linker
EAAAKEAAAKEAAAK

SEQ ID NO: 91 - protein, 15 aa, synthetic construct
  source 1..15: note = Linker
EAAAREAAAREAAAR

SEQ ID NO: 92 - protein, 15 aa, synthetic construct
  source 1..15: note = Linker
EGGGKEGGGKEGGGK

SEQ ID NO: 93 - protein, 15 aa, synthetic construct
  source 1..15: note = Linker
EGGGREGGGREGGGR

SEQ ID NO: 94 - protein, 15 aa, synthetic construct
  source 1..15: note = Linker
DAAARDAAARDAAAR

SEQ ID NO: 95 - protein, 15 aa, synthetic construct
  source 1..15: note = Linker
DAAAKDAAAKDAAAK

SEQ ID NO: 96 - protein, 15 aa, synthetic construct
  source 1..15: note = Linker
DGGGRDGGGRDGGGR

SEQ ID NO: 97 - protein, 15 aa, synthetic construct
  source 1..15: note = Linker
DGGGKDGGGKDGGGK

SEQ ID NO: 98 - protein, 4 aa, synthetic construct
  source 1..4: note = Linker
GGGS

SEQ ID NO: 99 - protein, 5 aa, synthetic construct
  source 1..5: note = Linker
GGGGG

SEQ ID NO: 100 - protein, 5 aa, synthetic construct
  source 1..5: note = Linker
GGGGS